European Patent Specification EP 3 597 221 B1, published August 30, 2023. Title: A agent for suppressing or decreasing photoperceptive sensitivity. Applicant: Osaka University Furukawa, Takahisa. The sequence listing filed with the application follows.

SEQUENCE LISTING (85 sequences)

SEQ ID NO: 1 - DNA, 4573 bp, Mus musculus
ggcttcgcgttctgggcagccttcagcgtgagcccttgccccgccctggttagtgtgaagcctgctggccaggcctgcgcagttgcggcggccggggaagatggtggaggacggcgcggaggagctggaggacttggtgcatttctccgtgtcggagttgcctagtcgcggctacggcgtcatggaggagatccggcggcagggcaagctatgcgacgtgacgctaaagattggggaccacaagttcagtgctcaccggatcgtcttagcggcctccatcccgtacttccatgctatgtttacgaacgacatgatggagtgcaagcaggatgagattgtaatgcagggaatggacccaagtgccctggaggctctcatcaactttgcttataatggcaaccttgctatcgaccagcagaatgtgcagtccctgctgatgggggcaagcttcctgcagctgcagagcatcaaagatgcttgctgcacgttcctccgagaaaggcttcaccccaaaaattgcctgggtgtgcgccagtttgccgagacgatgatgtgtgctgtgttgtacgatgcagccaacagcttcatccaccagcactttgtagaggtgtctctgtccgaagagttcctggccctgcccttggaagacgtgcttgagctggtgtcccgggatgagctgaatgtgaagtcagaggagcaggtttttgaagctgcattggcctgggtcaggtatgaccgggagcagaggggaccatgcctgcccgagctgctgtccaatatccgcctgcctctttgccggccccagttcttatcagatcgagtgcagcaagatgacctggtacggtgctgtcacaaatgcagggacctggtcgatgaagcaaaggactatcatctgatgccagagcgccggccccacctgccagctttcaggactcggccccgatgctgcacgtccatcgctgggctcatctacgctgtggggggcctcaactcagcaggtgattccctgaatgtggtggaagtgttcgaccctatcgccaatcgctgggaaaagtgccatcccatgacaacagcccgaagccgtgtgggtgtggctgtggtgaacgggctcctctatgctatcgggggatatgatggtcagttgcggctgagcaccgtggaggcctacaatcctgagacggacacatggacccgagtggggagcatgaatagcaagcgaagtgccatggggacagtcgtgctggatggacagatctacgtgtgtggaggctatgacggcaactcctccctcaactctgtggagacctactcacctgagacggacaagtggacagtggtgactccgatgagctcaaaccggagtgctgctggggtgacagtctttgagggcaggatatatgtgtcaggaggccacgatggcttgcagatcttcagcagtgtggaacactacaaccaccacacggccacctggcacccggcagccagcatgctcaacaagcgctgccgacacggagccgcctccctgggaagcaagatgtttgtctgtgggggctatgatggctctggcttcctcagtattgctgagatgtacagctctgtggcagaccagtggtgtctcatagtacccatgcacacacgccggagccgggtctccctcgtggccagctgtgggcgcctctatgcagtgggaggttacgatggacagtcaaacctaagctcagtggagatgtacgacccagagacggaccgctggacatttatggcccccatggcatgccacgaggggggggttggtgtgggctgcatccctcttctcaccatctaaggagaggatgggacgtggtgggctagggatctggtacaagcataggcgcttccttccaggggagagtcctctcagaagaggcagtggtggaccagaagacggggtgtaatgtgagcttgccagagggacagtttttccaggtgcttaagtcctctctcactgtgctgcccttgtgaccttaggttgtcaagatgcacagcacaggacaggagtccctctggggtcccacagccagtaacacggaagtgctttgctggtccaggcacacaggctccatccaagcccagcgaacacctgctgcagcactggcccagctcccccttgccacagggagcactcatgggcaggaggtcttccagccgagccttcccttctcctgcagccctgctgtggccgcttgggaagtgtgggtaaagctgggagagaagggacaccctggtgttgtcactgcctgtggtggtgcagctacagcagctagcatgctgcgagtgcacgggctctcccttcgacaggggcacagaggacttggcccctgtctccagcaagcagggagaacagaagtcttccccatgcctgattttttgggaatccagtgaggtctttctccacttgtccccaagaaacaggaagggaatggagatgctcgagagaaactggaggaaatggaaacaagaaaatgttgaagagaaactggaaggaaaaggcttgaagtgaacattttccacaggacggaaacagaaaagacactaaaaacaaacacacatttacatggagaaccatcaaccatgacaacagtggtgtccactcccacattcggatcccagggtcctacgtcctcctaaagcagtcggggtttcctctgaatcccacagtgtgtctgaaatcaggacattcttgactgacctgtagcaaggtgctcatggggtttggtctcctcacccacgtcagaggactttttaaatcataggcttagggagcgggttaaattactgccactcacctctgcccgagctcccaactgtcaccccatggttacctccctacaccacccagcgctcccacagatccccactcccacgtacatcctttccctttttggccagcaagaaacaacatgtctgcccagattcgcactcacccatccaccatccttgaataactctccctcatcacaacgcttccagagcacattgaccatttgtacctctaggacctaaccaggggcttgctcctaccagccatggaccagcttggtcaggtgactcgtcttccctgccattccgctattttccatccatttgccaaccctgggtgtccgtccaccttctctccagcaagatgggcctttacattcaagctacgaacgctggcgtcatggtataaaggcttacaaagaaatgtcttttgctgctgcaaggaagagattttctatttcttcccctgatcttggcaaatgacctcgtgaagagactcaatgctcctcctccctctggatgggaccttaccatagcacagaaggacccagagggagactgtctcttaccagtgcactgggcagtggggcagaccttcaactgccgctgccaaaatctgctttcctaaaatccttccagtagcgacgagaaggatataattgtttctagccccaaactgggtcttagggtccggtctgttccactgtccacctgattggtttcttgccctctgctgcctgcctggatcggcctagaagacggttcaggcggctctgggtgaagcctgcgggggcaggggggtggtccctttccccagaccatcaggtttcccagtgtgtgcaattgccatagattcagaaggaaggactcttgttccctgcaatgtaaagagccgggcctctgctctaagcacttgaaaataatgtttttatcttaaaagactgaacaatctggtaactgatacatcttaactaggctcccagtggagcgccagcatttcttcctgcccctcagtttgcctgctgaggtagactctaggggactatgggtcttggtttcctcttagtcctattaggaggggtgtatccacgctcctcttattaagtccttctgtgaatgtactgcccagcctcgactgtgaaggtgctgagaaccagtccgtgggctcccaggtgggcctcctgggtcctcacgatgcaagcagactgcatccctagagatgatacgccatctccccaccccccccgccaccccaccccggcctgctgctgccaggttaaccttcctgcctccactcccacctcctagtgtagacagtgtttccaagaaccatcaagtcagtgttttgatctaggctctgagcacacaagcgaacagaaacatttttatactcccctgtctgagggcgatggctgatctgtctcagtgtcagaactgtaggatcatgtgagaacaggcatcacccaaggacactggaaagaatgtagcaggaggtgggtccgacacgcctggtgggccatggggtctggccactgcacttcctcttctcctctctctctgggcttcaccagaggtcacaagcagaagagagctgaagcccagcctctgatggaactaagtaggaatcctgaccctcttcacccacagctatttcacgggaaacttttatttataggacgcatgtcttttgtgttgagaaaccaaagagaaataaagagaacacgcctaataaaaaaaaaaaaaaaaaaaaaaaaaaaaaaaaaaaaaaaaaaaa

SEQ ID NO: 2 - DNA, 1725 bp, Mus musculus
atggtggaggacggcgcggaggagctggaggacttggtgcatttctccgtgtcggagttgcctagtcgcggctacggcgtcatggaggagatccggcggcagggcaagctatgcgacgtgacgctaaagattggggaccacaagttcagtgctcaccggatcgtcttagcggcctccatcccgtacttccatgctatgtttacgaacgacatgatggagtgcaagcaggatgagattgtaatgcagggaatggacccaagtgccctggaggctctcatcaactttgcttataatggcaaccttgctatcgaccagcagaatgtgcagtccctgctgatgggggcaagcttcctgcagctgcagagcatcaaagatgcttgctgcacgttcctccgagaaaggcttcaccccaaaaattgcctgggtgtgcgccagtttgccgagacgatgatgtgtgctgtgttgtacgatgcagccaacagcttcatccaccagcactttgtagaggtgtctctgtccgaagagttcctggccctgcccttggaagacgtgcttgagctggtgtcccgggatgagctgaatgtgaagtcagaggagcaggtttttgaagctgcattggcctgggtcaggtatgaccgggagcagaggggaccatgcctgcccgagctgctgtccaatatccgcctgcctctttgccggccccagttcttatcagatcgagtgcagcaagatgacctggtacggtgctgtcacaaatgcagggacctggtcgatgaagcaaaggactatcatctgatgccagagcgccggccccacctgccagctttcaggactcggccccgatgctgcacgtccatcgctgggctcatctacgctgtggggggcctcaactcagcaggtgattccctgaatgtggtggaagtgttcgaccctatcgccaatcgctgggaaaagtgccatcccatgacaacagcccgaagccgtgtgggtgtggctgtggtgaacgggctcctctatgctatcgggggatatgatggtcagttgcggctgagcaccgtggaggcctacaatcctgagacggacacatggacccgagtggggagcatgaatagcaagcgaagtgccatggggacagtcgtgctggatggacagatctacgtgtgtggaggctatgacggcaactcctccctcaactctgtggagacctactcacctgagacggacaagtggacagtggtgactccgatgagctcaaaccggagtgctgctggggtgacagtctttgagggcaggatatatgtgtcaggaggccacgatggcttgcagatcttcagcagtgtggaacactacaaccaccacacggccacctggcacccggcagccagcatgctcaacaagcgctgccgacacggagccgcctccctgggaagcaagatgtttgtctgtgggggctatgatggctctggcttcctcagtattgctgagatgtacagctctgtggcagaccagtggtgtctcatagtacccatgcacacacgccggagccgggtctccctcgtggccagctgtgggcgcctctatgcagtgggaggttacgatggacagtcaaacctaagctcagtggagatgtacgacccagagacggaccgctggacatttatggcccccatggcatgccacgaggggggggttggtgtgggctgcatccctcttctcaccatctaa

SEQ ID NO: 3 - protein, 574 aa, Mus musculus
MVEDGAEELEDLVHFSVSELPSRGYGVMEEIRRQGKLCDVTLKIGDHKFSAHRIVLAASIPYFHAMFTNDMMECKQDEIVMQGMDPSALEALINFAYNGNLAIDQQNVQSLLMGASFLQLQSIKDACCTFLRERLHPKNCLGVRQFAETMMCAVLYDAANSFIHQHFVEVSLSEEFLALPLEDVLELVSRDELNVKSEEQVFEAALAWVRYDREQRGPCLPELLSNIRLPLCRPQFLSDRVQQDDLVRCCHKCRDLVDEAKDYHLMPERRPHLPAFRTRPRCCTSIAGLIYAVGGLNSAGDSLNVVEVFDPIANRWEKCHPMTTARSRVGVAVVNGLLYAIGGYDGQLRLSTVEAYNPETDTWTRVGSMNSKRSAMGTVVLDGQIYVCGGYDGNSSLNSVETYSPETDKWTVVTPMSSNRSAAGVTVFEGRIYVSGGHDGLQIFSSVEHYNHHTATWHPAASMLNKRCRHGAASLGSKMFVCGGYDGSGFLSIAEMYSSVADQWCLIVPMHTRRSRVSLVASCGRLYAVGGYDGQSNLSSVEMYDPETDRWTFMAPMACHEGGVGVGCIPLLTI

SEQ ID NO: 4 - DNA, 4538 bp, Mus musculus
cgcgttctgggcagccttcagcgtgagcccttgccccgccctggttagtgtgaagcctgctggccaggcctgcgcagttgcggcggccggggaagatggtggaggacggcgcggaggagctggaggacttggtgcatttctccgtgtcggagttgcctagtcgcggctacggcgtcatggaggagatccggcggcagggcaagctatgcgacgtgacgctaaagattggggaccacaagttcagtgctcaccggatcgtcttagcggcctccatcccgtacttccatgctatgtttacgaacgacatgatggagtgcaagcaggatgagattgtaatgcagggaatggacccaagtgccctggaggctctcatcaactttgcttataatggcaaccttgctatcgaccagcagaatgtgcagtccctgctgatgggggcaagcttcctgcagctgcagagcatcaaagatgcttgctgcacgttcctccgagaaaggcttcaccccaaaaattgcctgggtgtgcgccagtttgccgagacgatgatgtgtgctgtgttgtacgatgcagccaacagcttcatccaccagcactttgtagaggtgtctctgtccgaagagttcctggccctgcccttggaagacgtgcttgagctggtgtcccgggatgagctgaatgtgaagtcagaggagcaggtttttgaagctgcattggcctgggtcaggtatgaccgggagcagaggggaccatgcctgcccgagctgctgtccaatatccgcctgcctctttgccggccccagttcttatcagatcgagtgcagcaagatgacctggtacggtgctgtcacaaatgcagggacctggtcgatgaagcaaaggactatcatctgatgccagagcgccggccccacctgccagctttcaggactcggccccgatgctgcacgtccatcgctgggctcatctacgctgtggggggcctcaactcagcagcaaatttttatgcaggtgattccctgaatgtggtggaagtgttcgaccctatcgccaatcgctgggaaaagtgccatcccatgacaacagcccgaagccgtgtgggtgtggctgtggtgaacgggctcctctatgctatcgggggatatgatggtcagttgcggctgagcaccgtggaggcctacaatcctgagacggacacatggacccgagtggggagcatgaatagcaagcgaagtgccatggggacagtcgtgctggatggacagatctacgtgtgtggaggctatgacggcaactcctccctcaactctgtggagacctactcacctgagacggacaagtggacagtggtgactccgatgagctcaaaccggagtgctgctggggtgacagtctttgagggcaggatatatgtgtcaggaggccacgatggcttgcagatcttcagcagtgtggaacactacaaccaccacacggccacctggcacccggcagccagcatgctcaacaagcgctgccgacacggagccgcctccctgggaagcaagatgtttgtctgtgggggctatgatggctctggcttcctcagtattgctgagatgtacagctctgtggcagaccagtggtgtctcatagtacccatgcacacacgccggagccgggtctccctcgtggccagctgtgggcgcctctatgcagtgggaggttacgatggacagtcaaacctaagctcagtggagatgtacgacccagagacggaccgctggacatttatggcccccatggcatgccacgaggggggggttggtgtgggctgcatccctcttctcaccatctaaggagaggatgggacgtggtgggctagggatctggtacaagcataggcgcttccttccaggggagagtcctctcagaagaggcagtggtggaccagaagacggggtgtaatgtgagcttgccagagggacagtttttccaggtgcttaagtcctctctcactgtgctgcccttgtgaccttaggttgtcaagatgcacagcacaggacaggagtccctctggggtcccacagccagtaacacggaagtgctttgctggtccaggcacacaggctccatccaagcccagcgaacacctgctgcagcactggcccagctcccccttgccacagggagcactcatgggcaggaggtcttccagccgagccttcccttctcctgcagccctgctgtggccgcttgggaagtgtgggtaaagctgggagagaagggacaccctggtgttgtcactgcctgtggtggtgcagctacagcagctagcatgctgcgagtgcacgggctctcccttcgacaggggcacagaggacttggcccctgtctccagcaagcagggagaacagaagtcttccccatgcctgattttttgggaatccagtgaggtctttctccacttgtccccaagaaacaggaagggaatggagatgctcgagagaaactggaggaaatggaaacaagaaaatgttgaagagaaactggaaggaaaaggcttgaagtgaacattttccacaggacggaaacagaaaagacactaaaaacaaacacacatttacatggagaaccatcaaccatgacaacagtggtgtccactcccacattcggatcccagggtcctacgtcctcctaaagcagtcggggtttcctctgaatcccacagtgtgtctgaaatcaggacattcttgactgacctgtagcaaggtgctcatggggtttggtctcctcacccacgtcagaggactttttaaatcataggcttagggagcgggttaaattactgccactcacctctgcccgagctcccaactgtcaccccatggttacctccctacaccacccagcgctcccacagatccccactcccacgtacatcctttccctttttggccagcaagaaacaacatgtctgcccagattcgcactcacccatccaccatccttgaataactctccctcatcacaacgcttccagagcacattgaccatttgtacctctaggacctaaccaggggcttgctcctaccagccatggaccagcttggtcaggtgactcgtcttccctgccattccgctattttccatccatttgccaaccctgggtgtccgtccaccttctctccagcaagatgggcctttacattcaagctacgaacgctggcgtcatggtataaaggcttacaaagaaatgtcttttgctgctgcaaggaagagattttctatttcttcccctgatcttggcaaatgacctcgtgaagagactcaatgctcctcctccctctggatgggaccttaccatagcacagaaggacccagagggagactgtctcttaccagtgcactgggcagtggggcagaccttcaactgccgctgccaaaatctgctttcctaaaatccttccagtagcgacgagaaggatataattgtttctagccccaaactgggtcttagggtccggtctgttccactgtccacctgattggtttcttgccctctgctgcctgcctggatcggcctagaagacggttcaggcggctctgggtgaagcctgcgggggcaggggggtggtccctttccccagaccatcaggtttcccagtgtgtgcaattgccatagattcagaaggaaggactcttgttccctgcaatgtaaagagccgggcctctgctctaagcacttgaaaataatgtttttatcttaaaagactgaacaatctggtaactgatacatcttaactaggctcccagtggagcgccagcatttcttcctgcccctcagtttgcctgctgaggtagactctaggggactatgggtcttggtttcctcttagtcctattaggaggggtgtatccacgctcctcttattaagtccttctgtgaatgtactgcccagcctcgactgtgaaggtgctgagaaccagtccgtgggctcccaggtgggcctcctgggtcctcacgatgcaagcagactgcatccctagagatgatacgccatctccccaccccccccgccaccccaccccggcctgctgctgccaggttaaccttcctgcctccactcccacctcctagtgtagacagtgtttccaagaaccatcaagtcagtgttttgatctaggctctgagcacacaagcgaacagaaacatttttatactcccctgtctgagggcgatggctgatctgtctcagtgtcagaactgtaggatcatgtgagaacaggcatcacccaaggacactggaaagaatgtagcaggaggtgggtccgacacgcctggtgggccatggggtctggccactgcacttcctcttctcctctctctctgggcttcaccagaggtcacaagcagaagagagctgaagcccagcctctgatggaactaagtaggaatcctgaccctcttcacccacagctatttcacgggaaacttttatttataggacgcatgtcttttgtgttgagaaaccaaagagaaataaagagaacacgcctaa

SEQ ID NO: 5 - DNA, 1740 bp, Mus musculus
atggtggaggacggcgcggaggagctggaggacttggtgcatttctccgtgtcggagttgcctagtcgcggctacggcgtcatggaggagatccggcggcagggcaagctatgcgacgtgacgctaaagattggggaccacaagttcagtgctcaccggatcgtcttagcggcctccatcccgtacttccatgctatgtttacgaacgacatgatggagtgcaagcaggatgagattgtaatgcagggaatggacccaagtgccctggaggctctcatcaactttgcttataatggcaaccttgctatcgaccagcagaatgtgcagtccctgctgatgggggcaagcttcctgcagctgcagagcatcaaagatgcttgctgcacgttcctccgagaaaggcttcaccccaaaaattgcctgggtgtgcgccagtttgccgagacgatgatgtgtgctgtgttgtacgatgcagccaacagcttcatccaccagcactttgtagaggtgtctctgtccgaagagttcctggccctgcccttggaagacgtgcttgagctggtgtcccgggatgagctgaatgtgaagtcagaggagcaggtttttgaagctgcattggcctgggtcaggtatgaccgggagcagaggggaccatgcctgcccgagctgctgtccaatatccgcctgcctctttgccggccccagttcttatcagatcgagtgcagcaagatgacctggtacggtgctgtcacaaatgcagggacctggtcgatgaagcaaaggactatcatctgatgccagagcgccggccccacctgccagctttcaggactcggccccgatgctgcacgtccatcgctgggctcatctacgctgtggggggcctcaactcagcagcaaatttttatgcaggtgattccctgaatgtggtggaagtgttcgaccctatcgccaatcgctgggaaaagtgccatcccatgacaacagcccgaagccgtgtgggtgtggctgtggtgaacgggctcctctatgctatcgggggatatgatggtcagttgcggctgagcaccgtggaggcctacaatcctgagacggacacatggacccgagtggggagcatgaatagcaagcgaagtgccatggggacagtcgtgctggatggacagatctacgtgtgtggaggctatgacggcaactcctccctcaactctgtggagacctactcacctgagacggacaagtggacagtggtgactccgatgagctcaaaccggagtgctgctggggtgacagtctttgagggcaggatatatgtgtcaggaggccacgatggcttgcagatcttcagcagtgtggaacactacaaccaccacacggccacctggcacccggcagccagcatgctcaacaagcgctgccgacacggagccgcctccctgggaagcaagatgtttgtctgtgggggctatgatggctctggcttcctcagtattgctgagatgtacagctctgtggcagaccagtggtgtctcatagtacccatgcacacacgccggagccgggtctccctcgtggccagctgtgggcgcctctatgcagtgggaggttacgatggacagtcaaacctaagctcagtggagatgtacgacccagagacggaccgctggacatttatggcccccatggcatgccacgaggggggggttggtgtgggctgcatccctcttctcaccatctaa

SEQ ID NO: 6 - protein, 579 aa, Mus musculus
MVEDGAEELEDLVHFSVSELPSRGYGVMEEIRRQGKLCDVTLKIGDHKFSAHRIVLAASIPYFHAMFTNDMMECKQDEIVMQGMDPSALEALINFAYNGNLAIDQQNVQSLLMGASFLQLQSIKDACCTFLRERLHPKNCLGVRQFAETMMCAVLYDAANSFIHQHFVEVSLSEEFLALPLEDVLELVSRDELNVKSEEQVFEAALAWVRYDREQRGPCLPELLSNIRLPLCRPQFLSDRVQQDDLVRCCHKCRDLVDEAKDYHLMPERRPHLPAFRTRPRCCTSIAGLIYAVGGLNSAANFYAGDSLNVVEVFDPIANRWEKCHPMTTARSRVGVAVVNGLLYAIGGYDGQLRLSTVEAYNPETDTWTRVGSMNSKRSAMGTVVLDGQIYVCGGYDGNSSLNSVETYSPETDKWTVVTPMSSNRSAAGVTVFEGRIYVSGGHDGLQIFSSVEHYNHHTATWHPAASMLNKRCRHGAASLGSKMFVCGGYDGSGFLSIAEMYSSVADQWCLIVPMHTRRSRVSLVASCGRLYAVGGYDGQSNLSSVEMYDPETDRWTFMAPMACHEGGVGVGCIPLLTI

SEQ ID NO: 7 - DNA, 3165 bp, Mus musculus
cttcgcgttctgggcagccttcagcgtgagcccttgccccgccctggttagtgtgaagcctgctggccaggcctgcgcagttgcggcggccggggaagatggtggaggacggcgcggaggagctggaggacttggtgcatttctccgtgtcggagttgcctagtcgcggctacggcgtcatggaggagatccggcggcagggcaagctatgcgacgtgacgctaaagattggggaccacaagttcagtgctcaccggatcgtcttagcggcctccatcccgtacttccatgctatgtttacgaacgacatgatggagtgcaagcaggatgagattgtaatgcagggaatggacccaagtgccctggaggctctcatcaactttgcttataatggcaaccttgctatcgaccagcagaatgtgcagtccctgctgatgggggcaagcttcctgcagctgcagagcatcaaagatgcttgctgcacgttcctccgagaaaggcttcaccccaaaaattgcctgggtgtgcgccagtttgccgagacgatgatgtgtgctgtgttgtacgatgcagccaacagcttcatccaccagcactttgtagaggtgtctctgtccgaagagttcctggccctgcccttggaagacgtgcttgagctggtgtcccgggatgagctgaatgtgaagtcagaggagcagagtgagcatgtccaaaggagggaggagcttggcacaggaatggaggacacccatgtagccatctctagaacacaggtcagcagagaggtttttgaagctgcattggcctgggtcaggtatgaccgggagcagaggggaccatgcctgcccgagctgctgtccaatatccgcctgcctctttgccggccccagttcttatcagatcgagtgcagcaagatgacctggtacggtgctgtcacaaatgcagggacctggtcgatgaagcaaaggactatcatctgatgccagagcgccggccccacctgccagctttcaggactcggccccgatgctgcacgtccatcgctgggctcatctacgctgtggggggcctcaactcagcagcaaatttttatgcaggtgattccctgaatgtggtggaagtgttcgaccctatcgccaatcgctgggaaaagtgccatcccatgacaacagcccgaagccgtgtgggtgtggctgtggtgaacgggctcctctatgctatcgggggatatgatggtcagttgcggctgagcaccgtggaggcctacaatcctgagacggacacatggacccgagtggggagcatgaatagcaagcgaagtgccatggggacagtcgtgctggatggacagatctacgtgtgtggaggctatgacggcaactcctccctcaactctgtggagacctactcacctgagacggacaagtaaggctgacttatccccctgcctcagcttcttgagtgctgaaattacagatagaaactattatactcggcctaccttccccacctccaggcctttgtgcttgccaggcttccagcccccctccccccacccccactcccacctcttgtttagttttgctttgctttgttggagaaaaggtctcaacctcaggactctgatgagccacctcagccacagagacatgccgtggcacggagcttaaagcttctcctggctaggaagtgacttaacaatacttgcatgtagtcgatgtctacatccttggctaaatgtcagacacggtgatgcgcccctttgatccctttacttgaaggcagaggcaagtgtgtctccgtgagttcaaaaccagtctgctttatgtagtgcattctagactagccaaggctacaaagcaggacttggtctcaaaaaaacaaaacaaaaaaatatattttttaattccttgtttaagtgaaatttcatggttaaatttcaaaagagctaaagcaatggtggttcaatcccaagacttgaggtggaggcaggaggctcaggagttcgaggtgacatgaacccatttcaaataaacgaaaggctgagatgtttggaaacacttattccttggtcacgtcagtccactgtactggaagtgcaggtgcagatgctccttagaagcagataaggagcatctgcacagcttgttccacagcagtgaggcctgctgtgaaggactgtggggtcagagaaccccgggcagagttggtatctgtttcttcagagcctttgtcttgccaccacacatacgacattgcaaaagttctagaaaatctggcggtgaggaatcccgtttaaacttgcgttctctgtaacacccattacaatcgtgtaggatgcttttgtggaacactagaaacactggcaatgctggctgaattactcattctggtgtttgtatcctcccgtcttagataactgactgagcggatgggttgagccaactcatcagcacattctaaagccagtcttctgttgcctagcaactgactgcagctcttatcaagtagaaaggaggctggtcctccctggtgctcccttttggttatcctcaggtaggctggtcctccctggtgcctgcttttttttttatcagattgacaggttcctcctagcgctcagtttggtaggccatgagcgcactgtcactgtctttccttggaggtctgtgctgtgtctggagctcttatcatggtgtggggagcattcatcactctagggcaggggcacaaggtggactcaccagacagacagtgaggctgaggggatggcttacgtttataaaatatttgccctgcaagaatgaatccaaaaatgccaggcatgatagttcatgcttatagtcctggctgagaaggtggagacaggaggatccctcagagcttgctggcctgccagtctagcttaatagatgagctccaggccagtaagatcctgtgtctcagcacttgagagctacaacaggaggactccagtccaaagccagcccgagctacagaatgagagccttcctcagcaaacaaacagaaccaggcaggatggcacatgcctttaattccaggactaaggaggcagaggtagagggttcgaggctagccctgtctacagagttctaggacagccagggctacacagggctacaggtctcaaagaaagaaagaaa

SEQ ID NO: 8 - DNA, 1332 bp, Mus musculus
atggtggaggacggcgcggaggagctggaggacttggtgcatttctccgtgtcggagttgcctagtcgcggctacggcgtcatggaggagatccggcggcagggcaagctatgcgacgtgacgctaaagattggggaccacaagttcagtgctcaccggatcgtcttagcggcctccatcccgtacttccatgctatgtttacgaacgacatgatggagtgcaagcaggatgagattgtaatgcagggaatggacccaagtgccctggaggctctcatcaactttgcttataatggcaaccttgctatcgaccagcagaatgtgcagtccctgctgatgggggcaagcttcctgcagctgcagagcatcaaagatgcttgctgcacgttcctccgagaaaggcttcaccccaaaaattgcctgggtgtgcgccagtttgccgagacgatgatgtgtgctgtgttgtacgatgcagccaacagcttcatccaccagcactttgtagaggtgtctctgtccgaagagttcctggccctgcccttggaagacgtgcttgagctggtgtcccgggatgagctgaatgtgaagtcagaggagcagagtgagcatgtccaaaggagggaggagcttggcacaggaatggaggacacccatgtagccatctctagaacacaggtcagcagagaggtttttgaagctgcattggcctgggtcaggtatgaccgggagcagaggggaccatgcctgcccgagctgctgtccaatatccgcctgcctctttgccggccccagttcttatcagatcgagtgcagcaagatgacctggtacggtgctgtcacaaatgcagggacctggtcgatgaagcaaaggactatcatctgatgccagagcgccggccccacctgccagctttcaggactcggccccgatgctgcacgtccatcgctgggctcatctacgctgtggggggcctcaactcagcagcaaatttttatgcaggtgattccctgaatgtggtggaagtgttcgaccctatcgccaatcgctgggaaaagtgccatcccatgacaacagcccgaagccgtgtgggtgtggctgtggtgaacgggctcctctatgctatcgggggatatgatggtcagttgcggctgagcaccgtggaggcctacaatcctgagacggacacatggacccgagtggggagcatgaatagcaagcgaagtgccatggggacagtcgtgctggatggacagatctacgtgtgtggaggctatgacggcaactcctccctcaactctgtggagacctactcacctgagacggacaagtaa

SEQ ID NO: 9 - protein, 443 aa, Mus musculus
MVEDGAEELEDLVHFSVSELPSRGYGVMEEIRRQGKLCDVTLKIGDHKFSAHRIVLAASIPYFHAMFTNDMMECKQDEIVMQGMDPSALEALINFAYNGNLAIDQQNVQSLLMGASFLQLQSIKDACCTFLRERLHPKNCLGVRQFAETMMCAVLYDAANSFIHQHFVEVSLSEEFLALPLEDVLELVSRDELNVKSEEQSEHVQRREELGTGMEDTHVAISRTQVSREVFEAALAWVRYDREQRGPCLPELLSNIRLPLCRPQFLSDRVQQDDLVRCCHKCRDLVDEAKDYHLMPERRPHLPAFRTRPRCCTSIAGLIYAVGGLNSAANFYAGDSLNVVEVFDPIANRWEKCHPMTTARSRVGVAVVNGLLYAIGGYDGQLRLSTVEAYNPETDTWTRVGSMNSKRSAMGTVVLDGQIYVCGGYDGNSSLNSVETYSPETDK

SEQ ID NO: 10 - DNA, 4743 bp, Homo sapiens
gcggccgcggaggcccgtccgattgctgctccgcgctccgagcggctgtcggcgtgcgctatcgccccgccctggttagtgtctagccggccggcgaggcctgcgcagttgcagcggccggggaagatggtggaggacggcgcggaggagctggaggatctggtgcacttctccgtgtctgagttgcctagtcgcggctacggcgtcatggaggagatccggcggcagggcaagctgtgcgacgtgaccctcaagattggggaccacaaattcagtgcccaccggattgtcttagcagcctcgatcccgtatttccatgctatgtttacaaatgacatgatggagtgcaagcaggatgagattgtaatgcaaggaatggacccaagtgccctggaggctctgatcaactttgcctacaacggcaaccttgccattgaccagcaaaatgtccagtcattgctgatgggggcgagcttcctgcagctgcagagcatcaaagacgcctgctgcacattccttcgagaacggcttcacccaaaaaactgcctgggtgtgcgccagtttgctgagacaatgatgtgtgctgtgctgtacgacgctgccaacagcttcatccaccagcactttgtggaggtgtccatgtcagaagagttcctggccctgcccttggaagacgtgcttgagctggtgtctcgggatgagctgaatgtcaaatctgaggagcaggtctttgaagctgcattggcctgggtcagatacgaccgggagcagaggggtccctacctgcctgagctgctgtccaatatccgcctgcccctctgtcggccccagttcctttcagacagagtacagcaggatgacctggtgcgttgctgccacaaatgcagggacctggtagacgaagcaaaggactaccacctcatgccagagcgccggccccacctgccagctttcagaacccggccacgctgctgcacatccatcgctggacttatctacgctgtagggggcctcaactcagcaggtgattccctgaatgtggtggaagtgttcgaccccattgccaattgctgggagagatgccgtcccatgacaacagcccgcagccgcgttggcgtggctgtggtgaacgggcttctctatgccatcggaggatatgacggccagctacggctgagcactgtggaggcctacaacccggagacagacacatggaccagagtggggagcatgaatagcaagagaagtgccatggggacagtcgtgctggatgggcagatctacgtctgtgggggctacgatggcaactcttccctcagctccgtggagacctactcacctgagacggacaaatggacagtggtgacctcgatgagctcgaatcgcagtgctgctggggttacagtctttgagggcaggatatatgtgtcaggcggccatgatggtttgcagatcttcagcagtgtggaacactacaaccaccacacagccacctggcaccctgcagctggcatgctcaacaagcgctgccggcacggagccgcctccctggggagcaagatgtttgtctgcgggggctacgatggctctggcttcctcagcattgccgagatgtacagctctgtggcagaccagtggtgcctgattgtccccatgcacacgcgcaggagccgggtctccctggtggccagctgtgggcgcctctacgctgttgggggctacgacggacagtcaaacctaagctcagtggagatgtatgacccagagacagactgctggacattcatggcccccatggcgtgccatgagggaggggtcggtgtgggctgcatccctctcctcaccatctaaggcagaggatgggatgtggtggggcagggatctggtacagacataggcgcttccttccaggaacagtccctcaggagaggcagtggaccagaagagatggcgaaacgtgagctcgccggaggtacagtttttccaggtgcttaagccctcccccactgtgccacccttgtgaccttcaggcttgggtcatcaagatgcacagcatggaacacaagctcctctggatcctgcagctggtgacatggaactgttttctggtccacatgaacacaggctccatccaggcccagctcctacccaccgcctctctgtgggccagctgttcacagaaggccttccatctgatgctccccatcgcctgcttgctctccagccgagtctggccaatttgccatggggaggctgcagtgtccaagcctgctggaaactgggatgtagctggggacgaaaggacagacccaagcgttctccctgcctgagatggtgtggccacagcagtggaaggctgcacacaggcacattccttcttccacagtggggcaccaaggattctgtcctcattgctgggtaagcagggagaagagaagttttccccatgtctaattttgggatttcagtgaggccttttccatctgtccaggagaacagaagggaaaaaaagatacttgaaagaaactgaaggaaatttaaacaaagaaacacttgaaagaaactggaaagaaaaataatttttttatgtgaacaaattttgcaagaagaaaaaagcataaaagacactaacggcaaatctatgtttaaatggaaaatcgtctaactggagaagggcggtatccaccccacattcggatcccagggtcctgaggcctcgcattgagctgggggttccctctgagccccagtgtgtgtggaatcagtgcactcttgactgggcctgtagtaaggtgctcatggggtttgtcttctcacccaccatcagaggacttttaaaatcataggcgtagagagttagctatctgctgaattactgccactcttcttggtgggggctcctagctgtggctgggggctccaggcgcccctgtgattacctcctactgccaccatggcgctcattcagattccccactctcactaacattgcttccttttttgaccagcaggaaacagcaggtctggccagattctcacttgcccatcaatctcgttcttggatgatttccctcattgtgatgcttctggggcacgttgaccatatgcacctctagaacctaaccagggcttccttctaccagctgtgggcgggcttggtctggtaaccttgtctgctctgccattccactgctcctccatccactcgccaatcccaagagtctggcctccctccagccctgggcagactgaccagcaaggtggacctttacattcaagcacagctggcttttatgacataaagaactaaaggccgaaagaatctcttgctgctgcaaagaacagattttatatttcttcctctaatcttggcaaatgacctttaccttttggaaagatttcatattgcttcctcctccctggataggacctaatgtagcacagcgggactcaaagaggaggacattttctcttgccagtgcactgggcagtggggctgtccttcaactgctgctgccaaaattggttttctaaaattcttccagtagagactaaaagaagattcaattcctgtaacccaagactgagtcttagggctccagtctccacctgcttggtttcctatcctttgctgcctgcctggggtggcctggaagcctgttcagaaaggcacaatgtggagcctggggtgtctcccccaccccaggaccgtcaggtttaccagtgtgtgcaatcgccatgtattcagagggaagtacctttgttacctacaacttaggagctaggcctctgctacaagcacttgaaaatgatatttttatttttaacgtctcaacaatctgatatcggatgtcgtttaacctgggctcgtggtagggctccagcatttctccctccttcctggtttgcctgtaggggtagactcggaaggtgggtggggtgtgcatttcctgttaggagtgtatcagtgcttgtcttattataagcccctttcttttgtgaatttgaagtagcaccaacaagcctggattgtgaaggtattaagaatcggtctgtgggctactgagtgggtccttaggatactggcccagattttgccactgggtatggcagatcattttctaccatggcctgctgctcttgtagtggacttcctgagtccaatcccacctcctggtgtagaatttacactgctgcacctgaggtcgatgtttcaaagtaagatcaagccagtgttttgatctgggctctgagcacaagtcaggaaacaccaacatattcacactctcccagtaggttcctcagtccgatggtgaatggctattcgtaaatggctggtctggctctttggtgttggagcctttccaatagccccatgaaaagaagcatcacccaaggatattgtaaaaaggatgtaacaaggagatagggtagacattgtactcagtgggccttggggcctagcccagctctgagcagaggactgtggcattcactgtccttgagtgtttcaccttcttggataacacacgggccttctcttctggatttcatcagagattacagccagatgggggctgaagaccatcctcttgaccacagaggtgtgactgtgggaattcctcccaatttatggtttcccagaaaatcttagttccttttatttatagaatgcatgtcttttgtgttaagaaaccaaagagaaataaagagaacactcctaataaaaaaaaaaaaaaaaaa

SEQ ID NO: 11 - DNA, 1725 bp, Homo sapiens
atggtggaggacggcgcggaggagctggaggatctggtgcacttctccgtgtctgagttgcctagtcgcggctacggcgtcatggaggagatccggcggcagggcaagctgtgcgacgtgaccctcaagattggggaccacaaattcagtgcccaccggattgtcttagcagcctcgatcccgtatttccatgctatgtttacaaatgacatgatggagtgcaagcaggatgagattgtaatgcaaggaatggacccaagtgccctggaggctctgatcaactttgcctacaacggcaaccttgccattgaccagcaaaatgtccagtcattgctgatgggggcgagcttcctgcagctgcagagcatcaaagacgcctgctgcacattccttcgagaacggcttcacccaaaaaactgcctgggtgtgcgccagtttgctgagacaatgatgtgtgctgtgctgtacgacgctgccaacagcttcatccaccagcactttgtggaggtgtccatgtcagaagagttcctggccctgcccttggaagacgtgcttgagctggtgtctcgggatgagctgaatgtcaaatctgaggagcaggtctttgaagctgcattggcctgggtcagatacgaccgggagcagaggggtccctacctgcctgagctgctgtccaatatccgcctgcccctctgtcggccccagttcctttcagacagagtacagcaggatgacctggtgcgttgctgccacaaatgcagggacctggtagacgaagcaaaggactaccacctcatgccagagcgccggccccacctgccagctttcagaacccggccacgctgctgcacatccatcgctggacttatctacgctgtagggggcctcaactcagcaggtgattccctgaatgtggtggaagtgttcgaccccattgccaattgctgggagagatgccgtcccatgacaacagcccgcagccgcgttggcgtggctgtggtgaacgggcttctctatgccatcggaggatatgacggccagctacggctgagcactgtggaggcctacaacccggagacagacacatggaccagagtggggagcatgaatagcaagagaagtgccatggggacagtcgtgctggatgggcagatctacgtctgtgggggctacgatggcaactcttccctcagctccgtggagacctactcacctgagacggacaaatggacagtggtgacctcgatgagctcgaatcgcagtgctgctggggttacagtctttgagggcaggatatatgtgtcaggcggccatgatggtttgcagatcttcagcagtgtggaacactacaaccaccacacagccacctggcaccctgcagctggcatgctcaacaagcgctgccggcacggagccgcctccctggggagcaagatgtttgtctgcgggggctacgatggctctggcttcctcagcattgccgagatgtacagctctgtggcagaccagtggtgcctgattgtccccatgcacacgcgcaggagccgggtctccctggtggccagctgtgggcgcctctacgctgttgggggctacgacggacagtcaaacctaagctcagtggagatgtatgacccagagacagactgctggacattcatggcccccatggcgtgccatgagggaggggtcggtgtgggctgcatccctctcctcaccatctaa

SEQ ID NO: 12 - protein, 574 aa, Homo sapiens
MVEDGAEELEDLVHFSVSELPSRGYGVMEEIRRQGKLCDVTLKIGDHKFSAHRIVLAASIPYFHAMFTNDMMECKQDEIVMQGMDPSALEALINFAYNGNLAIDQQNVQSLLMGASFLQLQSIKDACCTFLRERLHPKNCLGVRQFAETMMCAVLYDAANSFIHQHFVEVSMSEEFLALPLEDVLELVSRDELNVKSEEQVFEAALAWVRYDREQRGPYLPELLSNIRLPLCRPQFLSDRVQQDDLVRCCHKCRDLVDEAKDYHLMPERRPHLPAFRTRPRCCTSIAGLIYAVGGLNSAGDSLNVVEVFDPIANCWERCRPMTTARSRVGVAVVNGLLYAIGGYDGQLRLSTVEAYNPETDTWTRVGSMNSKRSAMGTVVLDGQIYVCGGYDGNSSLSSVETYSPETDKWTVVTSMSSNRSAAGVTVFEGRIYVSGGHDGLQIFSSVEHYNHHTATWHPAAGMLNKRCRHGAASLGSKMFVCGGYDGSGFLSIAEMYSSVADQWCLIVPMHTRRSRVSLVASCGRLYAVGGYDGQSNLSSVEMYDPETDCWTFMAPMACHEGGVGVGCIPLLTI

SEQ ID NO: 13 - DNA, 4656 bp, Homo sapiens
ctgcgcagttgcagcggccggggaagatggtggaggacggcgcggaggagctggaggatctggtgcacttctccgtgtctgagttgcctagtcgcggctacggcgtcatggaggagatccggcggcagggcaagctgtgcgacgtgaccctcaagattggggaccacaaattcagtgcccaccggattgtcttagcagcctcgatcccgtatttccatgctatgtttacaaatgacatgatggagtgcaagcaggatgagattgtaatgcaaggaatggacccaagtgccctggaggctctgatcaactttgcctacaacggcaaccttgccattgaccagcaaaatgtccagtcattgctgatgggggcgagcttcctgcagctgcagagcatcaaagacgcctgctgcacattccttcgagaacggcttcacccaaaaaactgcctgggtgtgcgccagtttgctgagacaatgatgtgtgctgtgctgtacgacgctgccaacagcttcatccaccagcactttgtggaggtgtccatgtcagaagagttcctggccctgcccttggaagacgtgcttgagctggtgtctcgggatgagctgaatgtcaaatctgaggagcaggtctttgaagctgcattggcctgggtcagatacgaccgggagcagaggggtccctacctgcctgagctgctgtccaatatccgcctgcccctctgtcggccccagttcctttcagacagagtacagcaggatgacctggtgcgttgctgccacaaatgcagggacctggtagacgaagcaaaggactaccacctcatgccagagcgccggccccacctgccagctttcagaacccggccacgctgctgcacatccatcgctggacttatctacgctgtagggggcctcaactcagcagcaaatttttatgcaggtgattccctgaatgtggtggaagtgttcgaccccattgccaattgctgggagagatgccgtcccatgacaacagcccgcagccgcgttggcgtggctgtggtgaacgggcttctctatgccatcggaggatatgacggccagctacggctgagcactgtggaggcctacaacccggagacagacacatggaccagagtggggagcatgaatagcaagagaagctctgtctgtttcagtgccatggggacagtcgtgctggatgggcagatctacgtctgtgggggctacgatggcaactcttccctcagctccgtggagacctactcacctgagacggacaaatggacagtggtgacctcgatgagctcgaatcgcagtgctgctggggttacagtctttgagggcaggatatatgtgtcaggcggccatgatggtttgcagatcttcagcagtgtggaacactacaaccaccacacagccacctggcaccctgcagctggcatgctcaacaagcgctgccggcacggagccgcctccctggggagcaagatgtttgtctgcgggggctacgatggctctggcttcctcagcattgccgagatgtacagctctgtggcagaccagtggtgcctgattgtccccatgcacacgcgcaggagccgggtctccctggtggccagctgtgggcgcctctacgctgttgggggctacgacggacagtcaaacctaagctcagtggagatgtatgacccagagacagactgctggacattcatggcccccatggcgtgccatgagggaggggtcggtgtgggctgcatccctctcctcaccatctaaggcagaggatgggatgtggtggggcagggatctggtacagacataggcgcttccttccaggaacagtccctcaggagaggcagtggaccagaagagatggcgaaacgtgagctcgccggaggtacagtttttccaggtgcttaagccctcccccactgtgccacccttgtgaccttcaggcttgggtcatcaagatgcacagcatggaacacaagctcctctggatcctgcagctggtgacatggaactgttttctggtccacatgaacacaggctccatccaggcccagctcctacccaccgcctctctgtgggccagctgttcacagaaggccttccatctgatgctccccatcgcctgcttgctctccagccgagtctggccaatttgccatggggaggctgcagtgtccaagcctgctggaaactgggatgtagctggggacgaaaggacagacccaagcgttctccctgcctgagatggtgtggccacagcagtggaaggctgcacacaggcacattccttcttccacagtggggcaccaaggattctgtcctcattgctgggtaagcagggagaagagaagttttccccatgtctaattttgggatttcagtgaggccttttgatctgtccaggagaacagaagggaaaaaaagatacttgaaagaaactgaaggaaatttaaacaaagaaacacttgaaagaaactggaaagaaaaataatttttttatgtgaacaaattttgcaagaagaaaaaagcataaaagacactaacggcaaatctatgtttaaatggaaaatcgtctaactggagaagggcggtatccaccccacattcggatcccagggtcctgaggcctcgcattgagctgggggttccctctgagccccagtgtgtgtggaatcagtgcactcttgactgggcctgtagtaaggtgctcatggggtttgtcttctcacccaccatcagaggacttttaaaatcataggcgtagagagttaggctatctgctgaattactgccactcttcttggtgggggctcctagctgtggctgggggctccaggcgcccctgtgattacctcctactgccaccatggcgctcattcagattccccactctcactaacattgcttccttttttgaccagcaggaaacagcaggtctggccagattctcacttgcccatcaatctcgttcttggatgatttccctcattgtgatgcttctggggcacgttgaccatatgcacctctagaacctaaccagggcttccttctaccagctgtgggcgggcttggtctggtaaccttgtctgctctgccattccactgctcctccatccactcgccaatcccaagagtctggcctccctccagccctgggcagactgaccagcaaggtggacctttacattcaagcacagctggcttttatgacataaagaactaaaggccgaaagaatctcttgctgctgcaaagaacagattttatatttcttcctctaatcttggcaaatgacctttaccttttggaaagatttcatattgcttcctcctccctggataggacctaatgtagcacagcgggactcaaagaggaggacattttctcttgccagtgcactgggcagtggggctgtccttcaactgctgctgccaaaattggttttctaaaattcttccagtagagactaaaagaagattcaattcctgtaacccaagactgagtcttagggctccagtctccacctgcttggtttcctatcctttgctgcctgcctggggtggcctggaagcctgttcagaaaggcacaatgtggagcctggggtgtctcccccaccccaggaccgtcaggtttaccagtgtgtgcaatcgccatgtattcagagggaagtacctttgttacctacaacttaggagctaggcctctgctacaagcacttgaaaatgatatttttatttttaacgtctcaacaatctgatatcggatgtcgtttaacctgggctcgtggtagggctccagcatttctccctccttcctggtttgcctgtaggggtagactcggaaggtgggtggggtgtgcatttcctgttaggagtgtatcagtgcttgtcttattataagcccctttcttttgtgaatttgaagtagcaccaacaagcctggattgtgaaggtattaagaatcggtctgtgggctactgagtgggtccttaggatactggcccagattttgccactgggtatggcagatcattttctaccatggcctgctgctcttgtagtggacttcctgagtccaatcccacctcctggtgtagaatttacactgctgcacctgaggtcgatgtttcaaagtaagatcaagccagtgttttgatctgggctctgagcacaagtcaggaaacaccaacatattcacactctcccagtaggttcctcagtccgatggtgaatggctattcgtaaatggctggtctggctctttggtgttggagcctttccaatagccccatgaaaagaagcatcacccaaggatattgtaaaaaggatgtaacaaggagatagggtagacattgtactcagtgggccttggggcctagcccagctctgagcagaggactgtggcattcactgtccttgagtgtttcaccttcttggataacacacgggccttctcttctggatttcatcagagattacagccagatgggggctgaagaccatcctcttgaccacagaggtgtgactgtgggaattcctcccaatttatggtttcccagaaaatcttagttccttttatttatagaatgcatgtcttttgtgttaagaaaccaaagagaaataaagagaacactcctaata

SEQ ID NO: 14 - DNA, 1755 bp, Homo sapiens
atggtggaggacggcgcggaggagctggaggatctggtgcacttctccgtgtctgagttgcctagtcgcggctacggcgtcatggaggagatccggcggcagggcaagctgtgcgacgtgaccctcaagattggggaccacaaattcagtgcccaccggattgtcttagcagcctcgatcccgtatttccatgctatgtttacaaatgacatgatggagtgcaagcaggatgagattgtaatgcaaggaatggacccaagtgccctggaggctctgatcaactttgcctacaacggcaaccttgccattgaccagcaaaatgtccagtcattgctgatgggggcgagcttcctgcagctgcagagcatcaaagacgcctgctgcacattccttcgagaacggcttcacccaaaaaactgcctgggtgtgcgccagtttgctgagacaatgatgtgtgctgtgctgtacgacgctgccaacagcttcatccaccagcactttgtggaggtgtccatgtcagaagagttcctggccctgcccttggaagacgtgcttgagctggtgtctcgggatgagctgaatgtcaaatctgaggagcaggtctttgaagctgcattggcctgggtcagatacgaccgggagcagaggggtccctacctgcctgagctgctgtccaatatccgcctgcccctctgtcggccccagttcctttcagacagagtacagcaggatgacctggtgcgttgctgccacaaatgcagggacctggtagacgaagcaaaggactaccacctcatgccagagcgccggccccacctgccagctttcagaacccggccacgctgctgcacatccatcgctggacttatctacgctgtagggggcctcaactcagcagcaaatttttatgcaggtgattccctgaatgtggtggaagtgttcgaccccattgccaattgctgggagagatgccgtcccatgacaacagcccgcagccgcgttggcgtggctgtggtgaacgggcttctctatgccatcggaggatatgacggccagctacggctgagcactgtggaggcctacaacccggagacagacacatggaccagagtggggagcatgaatagcaagagaagctctgtctgtttcagtgccatggggacagtcgtgctggatgggcagatctacgtctgtgggggctacgatggcaactcttccctcagctccgtggagacctactcacctgagacggacaaatggacagtggtgacctcgatgagctcgaatcgcagtgctgctggggttacagtctttgagggcaggatatatgtgtcaggcggccatgatggtttgcagatcttcagcagtgtggaacactacaaccaccacacagccacctggcaccctgcagctggcatgctcaacaagcgctgccggcacggagccgcctccctggggagcaagatgtttgtctgcgggggctacgatggctctggcttcctcagcattgccgagatgtacagctctgtggcagaccagtggtgcctgattgtccccatgcacacgcgcaggagccgggtctccctggtggccagctgtgggcgcctctacgctgttgggggctacgacggacagtcaaacctaagctcagtggagatgtatgacccagagacagactgctggacattcatggcccccatggcgtgccatgagggaggggtcggtgtgggctgcatccctctcctcaccatctaa

SEQ ID NO: 15 - protein, 584 aa, Homo sapiens
MVEDGAEELEDLVHFSVSELPSRGYGVMEEIRRQGKLCDVTLKIGDHKFSAHRIVLAASIPYFHAMFTNDMMECKQDEIVMQGMDPSALEALINFAYNGNLAIDQQNVQSLLMGASFLQLQSIKDACCTFLRERLHPKNCLGVRQFAETMMCAVLYDAANSFIHQHFVEVSMSEEFLALPLEDVLELVSRDELNVKSEEQVFEAALAWVRYDREQRGPYLPELLSNIRLPLCRPQFLSDRVQQDDLVRCCHKCRDLVDEAKDYHLMPERRPHLPAFRTRPRCCTSIAGLIYAVGGLNSAANFYAGDSLNVVEVFDPIANCWERCRPMTTARSRVGVAVVNGLLYAIGGYDGQLRLSTVEAYNPETDTWTRVGSMNSKRSSVCFSAMGTVVLDGQIYVCGGYDGNSSLSSVETYSPETDKWTVVTSMSSNRSAAGVTVFEGRIYVSGGHDGLQIFSSVEHYNHHTATWHPAAGMLNKRCRHGAASLGSKMFVCGGYDGSGFLSIAEMYSSVADQWCLIVPMHTRRSRVSLVASCGRLYAVGGYDGQSNLSSVEMYDPETDCWTFMAPMACHEGGVGVGCIPLLTI

SEQ ID NO: 16 - DNA, 4641 bp, Homo sapiens
ctgcgcagttgcagcggccggggaagatggtggaggacggcgcggaggagctggaggatctggtgcacttctccgtgtctgagttgcctagtcgcggctacggcgtcatggaggagatccggcggcagggcaagctgtgcgacgtgaccctcaagattggggaccacaaattcagtgcccaccggattgtcttagcagcctcgatcccgtatttccatgctatgtttacaaatgacatgatggagtgcaagcaggatgagattgtaatgcaaggaatggacccaagtgccctggaggctctgatcaactttgcctacaacggcaaccttgccattgaccagcaaaatgtccagtcattgctgatgggggcgagcttcctgcagctgcagagcatcaaagacgcctgctgcacattccttcgagaacggcttcacccaaaaaactgcctgggtgtgcgccagtttgctgagacaatgatgtgtgctgtgctgtacgacgctgccaacagcttcatccaccagcactttgtggaggtgtccatgtcagaagagttcctggccctgcccttggaagacgtgcttgagctggtgtctcgggatgagctgaatgtcaaatctgaggagcaggtctttgaagctgcattggcctgggtcagatacgaccgggagcagaggggtccctacctgcctgagctgctgtccaatatccgcctgcccctctgtcggccccagttcctttcagacagagtacagcaggatgacctggtgcgttgctgccacaaatgcagggacctggtagacgaagcaaaggactaccacctcatgccagagcgccggccccacctgccagctttcagaacccggccacgctgctgcacatccatcgctggacttatctacgctgtagggggcctcaactcagcaggtgattccctgaatgtggtggaagtgttcgaccccattgccaattgctgggagagatgccgtcccatgacaacagcccgcagccgcgttggcgtggctgtggtgaacgggcttctctatgccatcggaggatatgacggccagctacggctgagcactgtggaggcctacaacccggagacagacacatggaccagagtggggagcatgaatagcaagagaagctctgtctgtttcagtgccatggggacagtcgtgctggatgggcagatctacgtctgtgggggctacgatggcaactcttccctcagctccgtggagacctactcacctgagacggacaaatggacagtggtgacctcgatgagctcgaatcgcagtgctgctggggttacagtctttgagggcaggatatatgtgtcaggcggccatgatggtttgcagatcttcagcagtgtggaacactacaaccaccacacagccacctggcaccctgcagctggcatgctcaacaagcgctgccggcacggagccgcctccctggggagcaagatgtttgtctgcgggggctacgatggctctggcttcctcagcattgccgagatgtacagctctgtggcagaccagtggtgcctgattgtccccatgcacacgcgcaggagccgggtctccctggtggccagctgtgggcgcctctacgctgttgggggctacgacggacagtcaaacctaagctcagtggagatgtatgacccagagacagactgctggacattcatggcccccatggcgtgccatgagggaggggtcggtgtgggctgcatccctctcctcaccatctaaggcagaggatgggatgtggtggggcagggatctggtacagacataggcgcttccttccaggaacagtccctcaggagaggcagtggaccagaagagatggcgaaacgtgagctcgccggaggtacagtttttccaggtgcttaagccctcccccactgtgccacccttgtgaccttcaggcttgggtcatcaagatgcacagcatggaacacaagctcctctggatcctgcagctggtgacatggaactgttttctggtccacatgaacacaggctccatccaggcccagctcctacccaccgcctctctgtgggccagctgttcacagaaggccttccatctgatgctccccatcgcctgcttgctctccagccgagtctggccaatttgccatggggaggctgcagtgtccaagcctgctggaaactgggatgtagctggggacgaaaggacagacccaagcgttctccctgcctgagatggtgtggccacagcagtggaaggctgcacacaggcacattccttcttccacagtggggcaccaaggattctgtcctcattgctgggtaagcagggagaagagaagttttccccatgtctaattttgggatttcagtgaggccttttgatctgtccaggagaacagaagggaaaaaaagatacttgaaagaaactgaaggaaatttaaacaaagaaacacttgaaagaaactggaaagaaaaataatttttttatgtgaacaaattttgcaagaagaaaaaagcataaaagacactaacggcaaatctatgtttaaatggaaaatcgtctaactggagaagggcggtatccaccccacattcggatcccagggtcctgaggcctcgcattgagctgggggttccctctgagccccagtgtgtgtggaatcagtgcactcttgactgggcctgtagtaaggtgctcatggggtttgtcttctcacccaccatcagaggacttttaaaatcataggcgtagagagttaggctatctgctgaattactgccactcttcttggtgggggctcctagctgtggctgggggctccaggcgcccctgtgattacctcctactgccaccatggcgctcattcagattccccactctcactaacattgcttccttttttgaccagcaggaaacagcaggtctggccagattctcacttgcccatcaatctcgttcttggatgatttccctcattgtgatgcttctggggcacgttgaccatatgcacctctagaacctaaccagggcttccttctaccagctgtgggcgggcttggtctggtaaccttgtctgctctgccattccactgctcctccatccactcgccaatcccaagagtctggcctccctccagccctgggcagactgaccagcaaggtggacctttacattcaagcacagctggcttttatgacataaagaactaaaggccgaaagaatctcttgctgctgcaaagaacagattttatatttcttcctctaatcttggcaaatgacctttaccttttggaaagatttcatattgcttcctcctccctggataggacctaatgtagcacagcgggactcaaagaggaggacattttctcttgccagtgcactgggcagtggggctgtccttcaactgctgctgccaaaattggttttctaaaattcttccagtagagactaaaagaagattcaattcctgtaacccaagactgagtcttagggctccagtctccacctgcttggtttcctatcctttgctgcctgcctggggtggcctggaagcctgttcagaaaggcacaatgtggagcctggggtgtctcccccaccccaggaccgtcaggtttaccagtgtgtgcaatcgccatgtattcagagggaagtacctttgttacctacaacttaggagctaggcctctgctacaagcacttgaaaatgatatttttatttttaacgtctcaacaatctgatatcggatgtcgtttaacctgggctcgtggtagggctccagcatttctccctccttcctggtttgcctgtaggggtagactcggaaggtgggtggggtgtgcatttcctgttaggagtgtatcagtgcttgtcttattataagcccctttcttttgtgaatttgaagtagcaccaacaagcctggattgtgaaggtattaagaatcggtctgtgggctactgagtgggtccttaggatactggcccagattttgccactgggtatggcagatcattttctaccatggcctgctgctcttgtagtggacttcctgagtccaatcccacctcctggtgtagaatttacactgctgcacctgaggtcgatgtttcaaagtaagatcaagccagtgttttgatctgggctctgagcacaagtcaggaaacaccaacatattcacactctcccagtaggttcctcagtccgatggtgaatggctattcgtaaatggctggtctggctctttggtgttggagcctttccaatagccccatgaaaagaagcatcacccaaggatattgtaaaaaggatgtaacaaggagatagggtagacattgtactcagtgggccttggggcctagcccagctctgagcagaggactgtggcattcactgtccttgagtgtttcaccttcttggataacacacgggccttctcttctggatttcatcagagattacagccagatgggggctgaagaccatcctcttgaccacagaggtgtgactgtgggaattcctcccaatttatggtttcccagaaaatcttagttccttttatttatagaatgcatgtcttttgtgttaagaaaccaaagagaaataaagagaacactcctaata

SEQ ID NO: 17 - DNA, 1740 bp, Homo sapiens
atggtggaggacggcgcggaggagctggaggatctggtgcacttctccgtgtctgagttgcctagtcgcggctacggcgtcatggaggagatccggcggcagggcaagctgtgcgacgtgaccctcaagattggggaccacaaattcagtgcccaccggattgtcttagcagcctcgatcccgtatttccatgctatgtttacaaatgacatgatggagtgcaagcaggatgagattgtaatgcaaggaatggacccaagtgccctggaggctctgatcaactttgcctacaacggcaaccttgccattgaccagcaaaatgtccagtcattgctgatgggggcgagcttcctgcagctgcagagcatcaaagacgcctgctgcacattccttcgagaacggcttcacccaaaaaactgcctgggtgtgcgccagtttgctgagacaatgatgtgtgctgtgctgtacgacgctgccaacagcttcatccaccagcactttgtggaggtgtccatgtcagaagagttcctggccctgcccttggaagacgtgcttgagctggtgtctcgggatgagctgaatgtcaaatctgaggagcaggtctttgaagctgcattggcctgggtcagatacgaccgggagcagaggggtccctacctgcctgagctgctgtccaatatccgcctgcccctctgtcggccccagttcctttcagacagagtacagcaggatgacctggtgcgttgctgccacaaatgcagggacctggtagacgaagcaaaggactaccacctcatgccagagcgccggccccacctgccagctttcagaacccggccacgctgctgcacatccatcgctggacttatctacgctgtagggggcctcaactcagcaggtgattccctgaatgtggtggaagtgttcgaccccattgccaattgctgggagagatgccgtcccatgacaacagcccgcagccgcgttggcgtggctgtggtgaacgggcttctctatgccatcggaggatatgacggccagctacggctgagcactgtggaggcctacaacccggagacagacacatggaccagagtggggagcatgaatagcaagagaagctctgtctgtttcagtgccatggggacagtcgtgctggatgggcagatctacgtctgtgggggctacgatggcaactcttccctcagctccgtggagacctactcacctgagacggacaaatggacagtggtgacctcgatgagctcgaatcgcagtgctgctggggttacagtctttgagggcaggatatatgtgtcaggcggccatgatggtttgcagatcttcagcagtgtggaacactacaaccaccacacagccacctggcaccctgcagctggcatgctcaacaagcgctgccggcacggagccgcctccctggggagcaagatgtttgtctgcgggggctacgatggctctggcttcctcagcattgccgagatgtacagctctgtggcagaccagtggtgcctgattgtccccatgcacacgcgcaggagccgggtctccctggtggccagctgtgggcgcctctacgctgttgggggctacgacggacagtcaaacctaagctcagtggagatgtatgacccagagacagactgctggacattcatggcccccatggcgtgccatgagggaggggtcggtgtgggctgcatccctctcctcaccatctaa

SEQ ID NO: 18 - protein, 579 aa, Homo sapiens
MVEDGAEELEDLVHFSVSELPSRGYGVMEEIRRQGKLCDVTLKIGDHKFSAHRIVLAASIPYFHAMFTNDMMECKQDEIVMQGMDPSALEALINFAYNGNLAIDQQNVQSLLMGASFLQLQSIKDACCTFLRERLHPKNCLGVRQFAETMMCAVLYDAANSFIHQHFVEVSMSEEFLALPLEDVLELVSRDELNVKSEEQVFEAALAWVRYDREQRGPYLPELLSNIRLPLCRPQFLSDRVQQDDLVRCCHKCRDLVDEAKDYHLMPERRPHLPAFRTRPRCCTSIAGLIYAVGGLNSAGDSLNVVEVFDPIANCWERCRPMTTARSRVGVAVVNGLLYAIGGYDGQLRLSTVEAYNPETDTWTRVGSMNSKRSSVCFSAMGTVVLDGQIYVCGGYDGNSSLSSVETYSPETDKWTVVTSMSSNRSAAGVTVFEGRIYVSGGHDGLQIFSSVEHYNHHTATWHPAAGMLNKRCRHGAASLGSKMFVCGGYDGSGFLSIAEMYSSVADQWCLIVPMHTRRSRVSLVASCGRLYAVGGYDGQSNLSSVEMYDPETDCWTFMAPMACHEGGVGVGCIPLLTI

SEQ ID NO: 19 - DNA, 4609 bp, Homo sapiens
ctgcgcagttgcagcggccggggaagatggtggaggacggcgcggaggagctggaggatctggtgcacttctccgtgtctgagttgcctagtcgcggctacggcgtcatggaggagatccggcggcagggcaagctgtgcgacgtgaccctcaagattggggaccacaaattcagtgcccaccggattgtcttagcagcctcgatcccgtatttccatgctatgtttacaaatgacatgatggagtgcaagcaggatgagattgtaatgcaaggaatggacccaagtgccctggaggctctgatcaactttgcctacaacggcaaccttgccattgaccagcaaaatgtccagtcattgctgatgggggcgagcttcctgcagctgcagagcatcaaagacgcctgctgcacattccttcgagaacggcttcacccaaaaaactgcctgggtgtgcgccagtttgctgagacaatgatgtgtgctgtgctgtacgacgctgccaacagcttcatccaccagcactttgtggaggtgtccatgtcagaagagttcctggccctgcccttggaagacgtgcttgagctggtgtctcgggatgagctgaatgtcaaatctgaggagcaggtctttgaagctgcattggcctgggtcagatacgaccgggagcagaggggtccctacctgcctgagctgctgtccaatatccgcctgcccctctgtcggccccagttcctttcagacagagtacagcaggatgacctggtgcgttgctgccacaaatgcagggacctggtagacgaagcaaaggactaccacctcatgccagagcgccggccccacctgccagctttcagaacccggccacgctgctgcacatccatcgctggacttatctacgctgtagggggcctcaactcagcagcaaatttttatgcaggtgattccctgaatgtggtggaagtgttcgaccccattgccaattgctgggagagatgccgtcccatgacaacagcccgcagccgcgttggcgtggctgtggtgaacgggcttctctatgccatcggaggatatgacggccagctacggctgagcactgtggaggcctacaacccggagacagacacatggaccagagtggggagcatgaatagcaagagaagtgccatggggacagtcgtgctggatgggcagatctacgtctgtgggggctacgatggcaactcttccctcagctccgtggagacctactcacctgagacggacaaatggacagtggtgacctcgatgagctcgaatcgcagtgctgctggggttacagtctttgagggcaggatatatgtgtcaggcggccatgatggtttgcagatcttcagcagtgtggaacactacaaccaccacacagccacctggcaccctgcagctggcatgctcaacaagcgctgccggcacggagccgcctccctggggagcaagatgtttgtctgcgggggctacgatggctctggcttcctcagcattgccgagatgtacagctctgtggcagaccagtggtgcctgattgtccccatgcacacgcgcaggagccgggtctccctggtggccagctgtgggcgcctctacgctgttgggggctacgacggacagtcaaacctaagctcagtggagatgtatgacccagagacagactgctggacattcatggcccccatggcgtgccatgagggaggggtcggtgtgggctgcatccctctcctcaccatctaaggcagaggatgggatgtggtggggcagggatctggtacagacataggcgcttccttccaggaacagtccctcaggagaggcagtggaccagaagagatggcgaaacgtgagctcgccggaggtacagtttttccaggtgcttaagccctcccccactgtgccacccttgtgaccttcaggcttgggtcatcaagatgcacagcatggaacacaagctcctctggatcctgcagctggtgacatggaactgttttctggtccacatgaacacaggctccatccaggcccagctcctacccaccgcctctctgtgggccagctgttcacagaaggccttccatctgatgctccccatcgcctgcttgctctccagccgagtctggccaatttgccatggggaggctgcagtgtccaagcctgctggaaactgggatgtagctggggacgaaaggacagacccaagcgttctccctgcctgagatggtgtggccacagcagtggaaggctgcacacaggcacattccttcttccacagtggggcaccaaggattctgtcctcattgctgggtaagcagggagaagagaagttttccccatgtctaattttgggatttcagtgaggccttttgatctgtccaggagaacagaagggaaaaaaagatacttgaaagaaactgaaggaaatttaaacaaagaaacacttgaaagaaactggaaagaaaaataatttttttatgtgaacaaattttgcaagaagaaaaaagcataaaagacactaacggcaaatctatgtttaaatggaaaatcgtctaactggagaagggcggtatccaccccacattcggatcccagggtcctgaggcctcgcattgagctgggggttccctctgagccccagtgtgtgtggaatcagtgcactcttgactgggcctgtagtaaggtgctcatggggtttgtcttctcacccaccatcagaggacttttaaaatcataggcgtagagagttaggctatctgctgaattactgccactcttcttggtgggggctcctagctgtggctgggggctccaggcgcccctgtgattacctcctactgccaccatggcgctcattcagattccccactctcactaacattgcttccttttttgaccagcaggaaacagcaggtctggccagattctcacttgcccatcaatctcgttcttggatgatttccctcattgtgatgcttctggggcacgttgaccatatgcacctctagaacctaaccagggcttccttctaccagctgtgggcgggcttggtctggtaaccttgtctgctctgccattccactgctcctccatccactcgccaatcccaagagtctggcctccctccagccctgggcagactgaccagcaaggtggacctttacattcaagcacagctggcttttatgacataaagaactaaaggccgaaagaatctcttgctgctgcaaagaacagattttatatttcttcctctaatcttggcaaatgacctttaccttttggaaagatttcatattgcttcctcctccctggataggacctaatgtagcacagcgggactcaaagaggaggacattttctcttgccagtgcactgggcagtggggctgtccttcaactgctgctgccaaaattggttttctaaaattcttccagtagagactaaaagaagattcaattcctgtaacccaagactgagtcttagggctccagtctccacctgcttggtttcctatcctttgctgcctgcctggggtggcctggaagcctgttcagaaaggcacaatgtggagcctggggtgtctcccccaccccaggaccgtcaggtttaccagtgtgtgcaatcgccatgtattcagagggaagtacctttgttacctacaacttaggagctaggcctctgctacaagcacttgaaaatgatatttttatttttaacgtctcaacaatctgatatcggatgtcgtttaacctgggctcgtggtagggctccagcatttctccctccttcctggtttgcctgtaggggtagactcggaaggtgggtggggtgtgcatttcctgttaggagtgtatcagtgcttgtcttattataagcccctttcttttgtgaatttgaagtagcaccaacaagcctggattgtgaaggtattaagaatcggtctgtgggctactgagtgggtccttaggatactggcccagattttgccactgggtatggcagatcattttctaccatggcctgctgctcttgtagtggacttcctgagtccaatcccacctcctggtgtagaatttacactgctgcacctgaggtcgatgtttcaaagtaagatcaagccagtgttttgatctgggctctgagcacaagtcaggaaacaccaacatattcacactctcccagtaggttcctcagtccgatggtgaatggctattcgtaaatggctggtctggctctttggtgttggagcctttccaatagccccatgaaaagaagcatcacccaaggatattgtaaaaaggatgtaacaaggagatagggtagacattgtactcagtgggccttggggcctagcccagctctgagcagaggactgtggcattcactgtccttgagtgtttcaccttcttggataacacacgggccttctcttctggatttcatcagagattacagccagatgggggctgaagaccatcctcttgaccacagaggtgtgactgtgggaattcctcccaatttatggtttcccagaaaatcttagttccttttatttatagaatgcatgtcttttgtgttaagaa

SEQ ID NO: 20 - DNA, 1740 bp, Homo sapiens
atggtggaggacggcgcggaggagctggaggatctggtgcacttctccgtgtctgagttgcctagtcgcggctacggcgtcatggaggagatccggcggcagggcaagctgtgcgacgtgaccctcaagattggggaccacaaattcagtgcccaccggattgtcttagcagcctcgatcccgtatttccatgctatgtttacaaatgacatgatggagtgcaagcaggatgagattgtaatgcaaggaatggacccaagtgccctggaggctctgatcaactttgcctacaacggcaaccttgccattgaccagcaaaatgtccagtcattgctgatgggggcgagcttcctgcagctgcagagcatcaaagacgcctgctgcacattccttcgagaacggcttcacccaaaaaactgcctgggtgtgcgccagtttgctgagacaatgatgtgtgctgtgctgtacgacgctgccaacagcttcatccaccagcactttgtggaggtgtccatgtcagaagagttcctggccctgcccttggaagacgtgcttgagctggtgtctcgggatgagctgaatgtcaaatctgaggagcaggtctttgaagctgcattggcctgggtcagatacgaccgggagcagaggggtccctacctgcctgagctgctgtccaatatccgcctgcccctctgtcggccccagttcctttcagacagagtacagcaggatgacctggtgcgttgctgccacaaatgcagggacctggtagacgaagcaaaggactaccacctcatgccagagcgccggccccacctgccagctttcagaacccggccacgctgctgcacatccatcgctggacttatctacgctgtagggggcctcaactcagcagcaaatttttatgcaggtgattccctgaatgtggtggaagtgttcgaccccattgccaattgctgggagagatgccgtcccatgacaacagcccgcagccgcgttggcgtggctgtggtgaacgggcttctctatgccatcggaggatatgacggccagctacggctgagcactgtggaggcctacaacccggagacagacacatggaccagagtggggagcatgaatagcaagagaagtgccatggggacagtcgtgctggatgggcagatctacgtctgtgggggctacgatggcaactcttccctcagctccgtggagacctactcacctgagacggacaaatggacagtggtgacctcgatgagctcgaatcgcagtgctgctggggttacagtctttgagggcaggatatatgtgtcaggcggccatgatggtttgcagatcttcagcagtgtggaacactacaaccaccacacagccacctggcaccctgcagctggcatgctcaacaagcgctgccggcacggagccgcctccctggggagcaagatgtttgtctgcgggggctacgatggctctggcttcctcagcattgccgagatgtacagctctgtggcagaccagtggtgcctgattgtccccatgcacacgcgcaggagccgggtctccctggtggccagctgtgggcgcctctacgctgttgggggctacgacggacagtcaaacctaagctcagtggagatgtatgacccagagacagactgctggacattcatggcccccatggcgtgccatgagggaggggtcggtgtgggctgcatccctctcctcaccatctaa

SEQ ID NO: 21 - protein, 579 aa, Homo sapiens
MVEDGAEELEDLVHFSVSELPSRGYGVMEEIRRQGKLCDVTLKIGDHKFSAHRIVLAASIPYFHAMFTNDMMECKQDEIVMQGMDPSALEALINFAYNGNLAIDQQNVQSLLMGASFLQLQSIKDACCTFLRERLHPKNCLGVRQFAETMMCAVLYDAANSFIHQHFVEVSMSEEFLALPLEDVLELVSRDELNVKSEEQVFEAALAWVRYDREQRGPYLPELLSNIRLPLCRPQFLSDRVQQDDLVRCCHKCRDLVDEAKDYHLMPERRPHLPAFRTRPRCCTSIAGLIYAVGGLNSAANFYAGDSLNVVEVFDPIANCWERCRPMTTARSRVGVAVVNGLLYAIGGYDGQLRLSTVEAYNPETDTWTRVGSMNSKRSAMGTVVLDGQIYVCGGYDGNSSLSSVETYSPETDKWTVVTSMSSNRSAAGVTVFEGRIYVSGGHDGLQIFSSVEHYNHHTATWHPAAGMLNKRCRHGAASLGSKMFVCGGYDGSGFLSIAEMYSSVADQWCLIVPMHTRRSRVSLVASCGRLYAVGGYDGQSNLSSVEMYDPETDCWTFMAPMACHEGGVGVGCIPLLTI

SEQ ID NO: 22 - DNA, 4519 bp, Homo sapiens
agttgcagcggccggggaagatggtggaggacggcgcggaggagctggaggatctggtgcacttctccgtgtctgagttgcctagtcgcggctacggcgtcatggaggagatccggcggcagggcaagctgtgcgacgtgaccctcaagtgccctggaggctctgatcaactttgcctacaacggcaaccttgccattgaccagcaaaatgtccagtcattgctgatgggggcgagcttcctgcagctgcagagcatcaaagacgcctgctgcacattccttcgagaacggcttcacccaaaaaactgcctgggtgtgcgccagtttgctgagacaatgatgtgtgctgtgctgtacgacgctgccaacagcttcatccaccagcactttgtggaggtgtccatgtcagaagagttcctggccctgcccttggaagacgtgcttgagctggtgtctcgggatgagctgaatgtcaaatctgaggagcaggtctttgaagctgcattggcctgggtcagatacgaccgggagcagaggggtccctacctgcctgagctgctgtccaatatccgcctgcccctctgtcggccccagttcctttcagacagagtacagcaggatgacctggtgcgttgctgccacaaatgcagggacctggtagacgaagcaaaggactaccacctcatgccagagcgccggccccacctgccagctttcagaacccggccacgctgctgcacatccatcgctggacttatctacgctgtagggggcctcaactcagcagcaaatttttatgcaggtgattccctgaatgtggtggaagtgttcgaccccattgccaattgctgggagagatgccgtcccatgacaacagcccgcagccgcgttggcgtggctgtggtgaacgggcttctctatgccatcggaggatatgacggccagctacggctgagcactgtggaggcctacaacccggagacagacacatggaccagagtggggagcatgaatagcaagagaagctctgtctgtttcagtgccatggggacagtcgtgctggatgggcagatctacgtctgtgggggctacgatggcaactcttccctcagctccgtggagacctactcacctgagacggacaaatggacagtggtgacctcgatgagctcgaatcgcagtgctgctggggttacagtctttgagggcaggatatatgtgtcaggcggccatgatggtttgcagatcttcagcagtgtggaacactacaaccaccacacagccacctggcaccctgcagctggcatgctcaacaagcgctgccggcacggagccgcctccctggggagcaagatgtttgtctgcgggggctacgatggctctggcttcctcagcattgccgagatgtacagctctgtggcagaccagtggtgcctgattgtccccatgcacacgcgcaggagccgggtctccctggtggccagctgtgggcgcctctacgctgttgggggctacgacggacagtcaaacctaagctcagtggagatgtatgacccagagacagactgctggacattcatggcccccatggcgtgccatgagggaggggtcggtgtgggctgcatccctctcctcaccatctaaggcagaggatgggatgtggtggggcagggatctggtacagacataggcgcttccttccaggaacagtccctcaggagaggcagtggaccagaagagatggcgaaacgtgagctcgccggaggtacagtttttccaggtgcttaagccctcccccactgtgccacccttgtgaccttcaggcttgggtcatcaagatgcacagcatggaacacaagctcctctggatcctgcagctggtgacatggaactgttttctggtccacatgaacacaggctccatccaggcccagctcctacccaccgcctctctgtgggccagctgttcacagaaggccttccatctgatgctccccatcgcctgcttgctctccagccgagtctggccaatttgccatggggaggctgcagtgtccaagcctgctggaaactgggatgtagctggggacgaaaggacagacccaagcgttctccctgcctgagatggtgtggccacagcagtggaaggctgcacacaggcacattccttcttccacagtggggcaccaaggattctgtcctcattgctgggtaagcagggagaagagaagttttccccatgtctaattttgggatttcagtgaggccttttgatctgtccaggagaacagaagggaaaaaaagatacttgaaagaaactgaaggaaatttaaacaaagaaacacttgaaagaaactggaaagaaaaataatttttttatgtgaacaaattttgcaagaagaaaaaagcataaaagacactaacggcaaatctatgtttaaatggaaaatcgtctaactggagaagggcggtatccaccccacattcggatcccagggtcctgaggcctcgcattgagctgggggttccctctgagccccagtgtgtgtggaatcagtgcactcttgactgggcctgtagtaaggtgctcatggggtttgtcttctcacccaccatcagaggacttttaaaatcataggcgtagagagttaggctatctgctgaattactgccactcttcttggtgggggctcctagctgtggctgggggctccaggcgcccctgtgattacctcctactgccaccatggcgctcattcagattccccactctcactaacattgcttccttttttgaccagcaggaaacagcaggtctggccagattctcacttgcccatcaatctcgttcttggatgatttccctcattgtgatgcttctggggcacgttgaccatatgcacctctagaacctaaccagggcttccttctaccagctgtgggcgggcttggtctggtaaccttgtctgctctgccattccactgctcctccatccactcgccaatcccaagagtctggcctccctccagccctgggcagactgaccagcaaggtggacctttacattcaagcacagctggcttttatgacataaagaactaaaggccgaaagaatctcttgctgctgcaaagaacagattttatatttcttcctctaatcttggcaaatgacctttaccttttggaaagatttcatattgcttcctcctccctggataggacctaatgtagcacagcgggactcaaagaggaggacattttctcttgccagtgcactgggcagtggggctgtccttcaactgctgctgccaaaattggttttctaaaattcttccagtagagactaaaagaagattcaattcctgtaacccaagactgagtcttagggctccagtctccacctgcttggtttcctatcctttgctgcctgcctggggtggcctggaagcctgttcagaaaggcacaatgtggagcctggggtgtctcccccaccccaggaccgtcaggtttaccagtgtgtgcaatcgccatgtattcagagggaagtacctttgttacctacaacttaggagctaggcctctgctacaagcacttgaaaatgatatttttatttttaacgtctcaacaatctgatatcggatgtcgtttaacctgggctcgtggtagggctccagcatttctccctccttcctggtttgcctgtaggggtagactcggaaggtgggtggggtgtgcatttcctgttaggagtgtatcagtgcttgtcttattataagcccctttcttttgtgaatttgaagtagcaccaacaagcctggattgtgaaggtattaagaatcggtctgtgggctactgagtgggtccttaggatactggcccagattttgccactgggtatggcagatcattttctaccatggcctgctgctcttgtagtggacttcctgagtccaatcccacctcctggtgtagaatttacactgctgcacctgaggtcgatgtttcaaagtaagatcaagccagtgttttgatctgggctctgagcacaagtcaggaaacaccaacatattcacactctcccagtaggttcctcagtccgatggtgaatggctattcgtaaatggctggtctggctctttggtgttggagcctttccaatagccccatgaaaagaagcatcacccaaggatattgtaaaaaggatgtaacaaggagatagggtagacattgtactcagtgggccttggggcctagcccagctctgagcagaggactgtggcattcactgtccttgagtgtttcaccttcttggataacacacgggccttctcttctggatttcatcagagattacagccagatgggggctgaagaccatcctcttgaccacagaggtgtgactgtgggaattcctcccaatttatggtttcccagaaaatcttagttccttttatttatagaatgcatgtcttttgtgttaagaaaccaaagagaaataaagagaacactcctaata

SEQ ID NO: 23 - DNA, 1419 bp, Homo sapiens
atgggggcgagcttcctgcagctgcagagcatcaaagacgcctgctgcacattccttcgagaacggcttcacccaaaaaactgcctgggtgtgcgccagtttgctgagacaatgatgtgtgctgtgctgtacgacgctgccaacagcttcatccaccagcactttgtggaggtgtccatgtcagaagagttcctggccctgcccttggaagacgtgcttgagctggtgtctcgggatgagctgaatgtcaaatctgaggagcaggtctttgaagctgcattggcctgggtcagatacgaccgggagcagaggggtccctacctgcctgagctgctgtccaatatccgcctgcccctctgtcggccccagttcctttcagacagagtacagcaggatgacctggtgcgttgctgccacaaatgcagggacctggtagacgaagcaaaggactaccacctcatgccagagcgccggccccacctgccagctttcagaacccggccacgctgctgcacatccatcgctggacttatctacgctgtagggggcctcaactcagcagcaaatttttatgcaggtgattccctgaatgtggtggaagtgttcgaccccattgccaattgctgggagagatgccgtcccatgacaacagcccgcagccgcgttggcgtggctgtggtgaacgggcttctctatgccatcggaggatatgacggccagctacggctgagcactgtggaggcctacaacccggagacagacacatggaccagagtggggagcatgaatagcaagagaagctctgtctgtttcagtgccatggggacagtcgtgctggatgggcagatctacgtctgtgggggctacgatggcaactcttccctcagctccgtggagacctactcacctgagacggacaaatggacagtggtgacctcgatgagctcgaatcgcagtgctgctggggttacagtctttgagggcaggatatatgtgtcaggcggccatgatggtttgcagatcttcagcagtgtggaacactacaaccaccacacagccacctggcaccctgcagctggcatgctcaacaagcgctgccggcacggagccgcctccctggggagcaagatgtttgtctgcgggggctacgatggctctggcttcctcagcattgccgagatgtacagctctgtggcagaccagtggtgcctgattgtccccatgcacacgcgcaggagccgggtctccctggtggccagctgtgggcgcctctacgctgttgggggctacgacggacagtcaaacctaagctcagtggagatgtatgacccagagacagactgctggacattcatggcccccatggcgtgccatgagggaggggtcggtgtgggctgcatccctctcctcaccatctaa

SEQ ID NO: 24 - protein, 472 aa, Homo sapiens
MGASFLQLQSIKDACCTFLRERLHPKNCLGVRQFAETMMCAVLYDAANSFIHQHFVEVSMSEEFLALPLEDVLELVSRDELNVKSEEQVFEAALAWVRYDREQRGPYLPELLSNIRLPLCRPQFLSDRVQQDDLVRCCHKCRDLVDEAKDYHLMPERRPHLPAFRTRPRCCTSIAGLIYAVGGLNSAANFYAGDSLNVVEVFDPIANCWERCRPMTTARSRVGVAVVNGLLYAIGGYDGQLRLSTVEAYNPETDTWTRVGSMNSKRSSVCFSAMGTVVLDGQIYVCGGYDGNSSLSSVETYSPETDKWTVVTSMSSNRSAAGVTVFEGRIYVSGGHDGLQIFSSVEHYNHHTATWHPAAGMLNKRCRHGAASLGSKMFVCGGYDGSGFLSIAEMYSSVADQWCLIVPMHTRRSRVSLVASCGRLYAVGGYDGQSNLSSVEMYDPETDCWTFMAPMACHEGGVGVGCIPLLTI

SEQ ID NO: 25 - DNA, 4504 bp, Homo sapiens
agttgcagcggccggggaagatggtggaggacggcgcggaggagctggaggatctggtgcacttctccgtgtctgagttgcctagtcgcggctacggcgtcatggaggagatccggcggcagggcaagctgtgcgacgtgaccctcaagtgccctggaggctctgatcaactttgcctacaacggcaaccttgccattgaccagcaaaatgtccagtcattgctgatgggggcgagcttcctgcagctgcagagcatcaaagacgcctgctgcacattccttcgagaacggcttcacccaaaaaactgcctgggtgtgcgccagtttgctgagacaatgatgtgtgctgtgctgtacgacgctgccaacagcttcatccaccagcactttgtggaggtgtccatgtcagaagagttcctggccctgcccttggaagacgtgcttgagctggtgtctcgggatgagctgaatgtcaaatctgaggagcaggtctttgaagctgcattggcctgggtcagatacgaccgggagcagaggggtccctacctgcctgagctgctgtccaatatccgcctgcccctctgtcggccccagttcctttcagacagagtacagcaggatgacctggtgcgttgctgccacaaatgcagggacctggtagacgaagcaaaggactaccacctcatgccagagcgccggccccacctgccagctttcagaacccggccacgctgctgcacatccatcgctggacttatctacgctgtagggggcctcaactcagcagcaaatttttatgcaggtgattccctgaatgtggtggaagtgttcgaccccattgccaattgctgggagagatgccgtcccatgacaacagcccgcagccgcgttggcgtggctgtggtgaacgggcttctctatgccatcggaggatatgacggccagctacggctgagcactgtggaggcctacaacccggagacagacacatggaccagagtggggagcatgaatagcaagagaagtgccatggggacagtcgtgctggatgggcagatctacgtctgtgggggctacgatggcaactcttccctcagctccgtggagacctactcacctgagacggacaaatggacagtggtgacctcgatgagctcgaatcgcagtgctgctggggttacagtctttgagggcaggatatatgtgtcaggcggccatgatggtttgcagatcttcagcagtgtggaacactacaaccaccacacagccacctggcaccctgcagctggcatgctcaacaagcgctgccggcacggagccgcctccctggggagcaagatgtttgtctgcgggggctacgatggctctggcttcctcagcattgccgagatgtacagctctgtggcagaccagtggtgcctgattgtccccatgcacacgcgcaggagccgggtctccctggtggccagctgtgggcgcctctacgctgttgggggctacgacggacagtcaaacctaagctcagtggagatgtatgacccagagacagactgctggacattcatggcccccatggcgtgccatgagggaggggtcggtgtgggctgcatccctctcctcaccatctaaggcagaggatgggatgtggtggggcagggatctggtacagacataggcgcttccttccaggaacagtccctcaggagaggcagtggaccagaagagatggcgaaacgtgagctcgccggaggtacagtttttccaggtgcttaagccctcccccactgtgccacccttgtgaccttcaggcttgggtcatcaagatgcacagcatggaacacaagctcctctggatcctgcagctggtgacatggaactgttttctggtccacatgaacacaggctccatccaggcccagctcctacccaccgcctctctgtgggccagctgttcacagaaggccttccatctgatgctccccatcgcctgcttgctctccagccgagtctggccaatttgccatggggaggctgcagtgtccaagcctgctggaaactgggatgtagctggggacgaaaggacagacccaagcgttctccctgcctgagatggtgtggccacagcagtggaaggctgcacacaggcacattccttcttccacagtggggcaccaaggattctgtcctcattgctgggtaagcagggagaagagaagttttccccatgtctaattttgggatttcagtgaggccttttgatctgtccaggagaacagaagggaaaaaaagatacttgaaagaaactgaaggaaatttaaacaaagaaacacttgaaagaaactggaaagaaaaataatttttttatgtgaacaaattttgcaagaagaaaaaagcataaaagacactaacggcaaatctatgtttaaatggaaaatcgtctaactggagaagggcggtatccaccccacattcggatcccagggtcctgaggcctcgcattgagctgggggttccctctgagccccagtgtgtgtggaatcagtgcactcttgactgggcctgtagtaaggtgctcatggggtttgtcttctcacccaccatcagaggacttttaaaatcataggcgtagagagttaggctatctgctgaattactgccactcttcttggtgggggctcctagctgtggctgggggctccaggcgcccctgtgattacctcctactgccaccatggcgctcattcagattccccactctcactaacattgcttccttttttgaccagcaggaaacagcaggtctggccagattctcacttgcccatcaatctcgttcttggatgatttccctcattgtgatgcttctggggcacgttgaccatatgcacctctagaacctaaccagggcttccttctaccagctgtgggcgggcttggtctggtaaccttgtctgctctgccattccactgctcctccatccactcgccaatcccaagagtctggcctccctccagccctgggcagactgaccagcaaggtggacctttacattcaagcacagctggcttttatgacataaagaactaaaggccgaaagaatctcttgctgctgcaaagaacagattttatatttcttcctctaatcttggcaaatgacctttaccttttggaaagatttcatattgcttcctcctccctggataggacctaatgtagcacagcgggactcaaagaggaggacattttctcttgccagtgcactgggcagtggggctgtccttcaactgctgctgccaaaattggttttctaaaattcttccagtagagactaaaagaagattcaattcctgtaacccaagactgagtcttagggctccagtctccacctgcttggtttcctatcctttgctgcctgcctggggtggcctggaagcctgttcagaaaggcacaatgtggagcctggggtgtctcccccaccccaggaccgtcaggtttaccagtgtgtgcaatcgccatgtattcagagggaagtacctttgttacctacaacttaggagctaggcctctgctacaagcacttgaaaatgatatttttatttttaacgtctcaacaatctgatatcggatgtcgtttaacctgggctcgtggtagggctccagcatttctccctccttcctggtttgcctgtaggggtagactcggaaggtgggtggggtgtgcatttcctgttaggagtgtatcagtgcttgtcttattataagcccctttcttttgtgaatttgaagtagcaccaacaagcctggattgtgaaggtattaagaatcggtctgtgggctactgagtgggtccttaggatactggcccagattttgccactgggtatggcagatcattttctaccatggcctgctgctcttgtagtggacttcctgagtccaatcccacctcctggtgtagaatttacactgctgcacctgaggtcgatgtttcaaagtaagatcaagccagtgttttgatctgggctctgagcacaagtcaggaaacaccaacatattcacactctcccagtaggttcctcagtccgatggtgaatggctattcgtaaatggctggtctggctctttggtgttggagcctttccaatagccccatgaaaagaagcatcacccaaggatattgtaaaaaggatgtaacaaggagatagggtagacattgtactcagtgggccttggggcctagcccagctctgagcagaggactgtggcattcactgtccttgagtgtttcaccttcttggataacacacgggccttctcttctggatttcatcagagattacagccagatgggggctgaagaccatcctcttgaccacagaggtgtgactgtgggaattcctcccaatttatggtttcccagaaaatcttagttccttttatttatagaatgcatgtcttttgtgttaagaaaccaaagagaaataaagagaacactcctaata

SEQ ID NO: 26 - DNA, 1404 bp, Homo sapiens
atgggggcgagcttcctgcagctgcagagcatcaaagacgcctgctgcacattccttcgagaacggcttcacccaaaaaactgcctgggtgtgcgccagtttgctgagacaatgatgtgtgctgtgctgtacgacgctgccaacagcttcatccaccagcactttgtggaggtgtccatgtcagaagagttcctggccctgcccttggaagacgtgcttgagctggtgtctcgggatgagctgaatgtcaaatctgaggagcaggtctttgaagctgcattggcctgggtcagatacgaccgggagcagaggggtccctacctgcctgagctgctgtccaatatccgcctgcccctctgtcggccccagttcctttcagacagagtacagcaggatgacctggtgcgttgctgccacaaatgcagggacctggtagacgaagcaaaggactaccacctcatgccagagcgccggccccacctgccagctttcagaacccggccacgctgctgcacatccatcgctggacttatctacgctgtagggggcctcaactcagcagcaaatttttatgcaggtgattccctgaatgtggtggaagtgttcgaccccattgccaattgctgggagagatgccgtcccatgacaacagcccgcagccgcgttggcgtggctgtggtgaacgggcttctctatgccatcggaggatatgacggccagctacggctgagcactgtggaggcctacaacccggagacagacacatggaccagagtggggagcatgaatagcaagagaagtgccatggggacagtcgtgctggatgggcagatctacgtctgtgggggctacgatggcaactcttccctcagctccgtggagacctactcacctgagacggacaaatggacagtggtgacctcgatgagctcgaatcgcagtgctgctggggttacagtctttgagggcaggatatatgtgtcaggcggccatgatggtttgcagatcttcagcagtgtggaacactacaaccaccacacagccacctggcaccctgcagctggcatgctcaacaagcgctgccggcacggagccgcctccctggggagcaagatgtttgtctgcgggggctacgatggctctggcttcctcagcattgccgagatgtacagctctgtggcagaccagtggtgcctgattgtccccatgcacacgcgcaggagccgggtctccctggtggccagctgtgggcgcctctacgctgttgggggctacgacggacagtcaaacctaagctcagtggagatgtatgacccagagacagactgctggacattcatggcccccatggcgtgccatgagggaggggtcggtgtgggctgcatccctctcctcaccatctaa

SEQ ID NO: 27 - protein, 467 aa, Homo sapiens
MGASFLQLQSIKDACCTFLRERLHPKNCLGVRQFAETMMCAVLYDAANSFIHQHFVEVSMSEEFLALPLEDVLELVSRDELNVKSEEQVFEAALAWVRYDREQRGPYLPELLSNIRLPLCRPQFLSDRVQQDDLVRCCHKCRDLVDEAKDYHLMPERRPHLPAFRTRPRCCTSIAGLIYAVGGLNSAANFYAGDSLNVVEVFDPIANCWERCRPMTTARSRVGVAVVNGLLYAIGGYDGQLRLSTVEAYNPETDTWTRVGSMNSKRSAMGTVVLDGQIYVCGGYDGNSSLSSVETYSPETDKWTVVTSMSSNRSAAGVTVFEGRIYVSGGHDGLQIFSSVEHYNHHTATWHPAAGMLNKRCRHGAASLGSKMFVCGGYDGSGFLSIAEMYSSVADQWCLIVPMHTRRSRVSLVASCGRLYAVGGYDGQSNLSSVEMYDPETDCWTFMAPMACHEGGVGVGCIPLLTI

SEQ ID NO: 28 - DNA, 4489 bp, Homo sapiens
agttgcagcggccggggaagatggtggaggacggcgcggaggagctggaggatctggtgcacttctccgtgtctgagttgcctagtcgcggctacggcgtcatggaggagatccggcggcagggcaagctgtgcgacgtgaccctcaagtgccctggaggctctgatcaactttgcctacaacggcaaccttgccattgaccagcaaaatgtccagtcattgctgatgggggcgagcttcctgcagctgcagagcatcaaagacgcctgctgcacattccttcgagaacggcttcacccaaaaaactgcctgggtgtgcgccagtttgctgagacaatgatgtgtgctgtgctgtacgacgctgccaacagcttcatccaccagcactttgtggaggtgtccatgtcagaagagttcctggccctgcccttggaagacgtgcttgagctggtgtctcgggatgagctgaatgtcaaatctgaggagcaggtctttgaagctgcattggcctgggtcagatacgaccgggagcagaggggtccctacctgcctgagctgctgtccaatatccgcctgcccctctgtcggccccagttcctttcagacagagtacagcaggatgacctggtgcgttgctgccacaaatgcagggacctggtagacgaagcaaaggactaccacctcatgccagagcgccggccccacctgccagctttcagaacccggccacgctgctgcacatccatcgctggacttatctacgctgtagggggcctcaactcagcaggtgattccctgaatgtggtggaagtgttcgaccccattgccaattgctgggagagatgccgtcccatgacaacagcccgcagccgcgttggcgtggctgtggtgaacgggcttctctatgccatcggaggatatgacggccagctacggctgagcactgtggaggcctacaacccggagacagacacatggaccagagtggggagcatgaatagcaagagaagtgccatggggacagtcgtgctggatgggcagatctacgtctgtgggggctacgatggcaactcttccctcagctccgtggagacctactcacctgagacggacaaatggacagtggtgacctcgatgagctcgaatcgcagtgctgctggggttacagtctttgagggcaggatatatgtgtcaggcggccatgatggtttgcagatcttcagcagtgtggaacactacaaccaccacacagccacctggcaccctgcagctggcatgctcaacaagcgctgccggcacggagccgcctccctggggagcaagatgtttgtctgcgggggctacgatggctctggcttcctcagcattgccgagatgtacagctctgtggcagaccagtggtgcctgattgtccccatgcacacgcgcaggagccgggtctccctggtggccagctgtgggcgcctctacgctgttgggggctacgacggacagtcaaacctaagctcagtggagatgtatgacccagagacagactgctggacattcatggcccccatggcgtgccatgagggaggggtcggtgtgggctgcatccctctcctcaccatctaaggcagaggatgggatgtggtggggcagggatctggtacagacataggcgcttccttccaggaacagtccctcaggagaggcagtggaccagaagagatggcgaaacgtgagctcgccggaggtacagtttttccaggtgcttaagccctcccccactgtgccacccttgtgaccttcaggcttgggtcatcaagatgcacagcatggaacacaagctcctctggatcctgcagctggtgacatggaactgttttctggtccacatgaacacaggctccatccaggcccagctcctacccaccgcctctctgtgggccagctgttcacagaaggccttccatctgatgctccccatcgcctgcttgctctccagccgagtctggccaatttgccatggggaggctgcagtgtccaagcctgctggaaactgggatgtagctggggacgaaaggacagacccaagcgttctccctgcctgagatggtgtggccacagcagtggaaggctgcacacaggcacattccttcttccacagtggggcaccaaggattctgtcctcattgctgggtaagcagggagaagagaagttttccccatgtctaattttgggatttcagtgaggccttttgatctgtccaggagaacagaagggaaaaaaagatacttgaaagaaactgaaggaaatttaaacaaagaaacacttgaaagaaactggaaagaaaaataatttttttatgtgaacaaattttgcaagaagaaaaaagcataaaagacactaacggcaaatctatgtttaaatggaaaatcgtctaactggagaagggcggtatccaccccacattcggatcccagggtcctgaggcctcgcattgagctgggggttccctctgagccccagtgtgtgtggaatcagtgcactcttgactgggcctgtagtaaggtgctcatggggtttgtcttctcacccaccatcagaggacttttaaaatcataggcgtagagagttaggctatctgctgaattactgccactcttcttggtgggggctcctagctgtggctgggggctccaggcgcccctgtgattacctcctactgccaccatggcgctcattcagattccccactctcactaacattgcttccttttttgaccagcaggaaacagcaggtctggccagattctcacttgcccatcaatctcgttcttggatgatttccctcattgtgatgcttctggggcacgttgaccatatgcacctctagaacctaaccagggcttccttctaccagctgtgggcgggcttggtctggtaaccttgtctgctctgccattccactgctcctccatccactcgccaatcccaagagtctggcctccctccagccctgggcagactgaccagcaaggtggacctttacattcaagcacagctggcttttatgacataaagaactaaaggccgaaagaatctcttgctgctgcaaagaacagattttatatttcttcctctaatcttggcaaatgacctttaccttttggaaagatttcatattgcttcctcctccctggataggacctaatgtagcacagcgggactcaaagaggaggacattttctcttgccagtgcactgggcagtggggctgtccttcaactgctgctgccaaaattggttttctaaaattcttccagtagagactaaaagaagattcaattcctgtaacccaagactgagtcttagggctccagtctccacctgcttggtttcctatcctttgctgcctgcctggggtggcctggaagcctgttcagaaaggcacaatgtggagcctggggtgtctcccccaccccaggaccgtcaggtttaccagtgtgtgcaatcgccatgtattcagagggaagtacctttgttacctacaacttaggagctaggcctctgctacaagcacttgaaaatgatatttttatttttaacgtctcaacaatctgatatcggatgtcgtttaacctgggctcgtggtagggctccagcatttctccctccttcctggtttgcctgtaggggtagactcggaaggtgggtggggtgtgcatttcctgttaggagtgtatcagtgcttgtcttattataagcccctttcttttgtgaatttgaagtagcaccaacaagcctggattgtgaaggtattaagaatcggtctgtgggctactgagtgggtccttaggatactggcccagattttgccactgggtatggcagatcattttctaccatggcctgctgctcttgtagtggacttcctgagtccaatcccacctcctggtgtagaatttacactgctgcacctgaggtcgatgtttcaaagtaagatcaagccagtgttttgatctgggctctgagcacaagtcaggaaacaccaacatattcacactctcccagtaggttcctcagtccgatggtgaatggctattcgtaaatggctggtctggctctttggtgttggagcctttccaatagccccatgaaaagaagcatcacccaaggatattgtaaaaaggatgtaacaaggagatagggtagacattgtactcagtgggccttggggcctagcccagctctgagcagaggactgtggcattcactgtccttgagtgtttcaccttcttggataacacacgggccttctcttctggatttcatcagagattacagccagatgggggctgaagaccatcctcttgaccacagaggtgtgactgtgggaattcctcccaatttatggtttcccagaaaatcttagttccttttatttatagaatgcatgtcttttgtgttaagaaaccaaagagaaataaagagaacactcctaata

SEQ ID NO: 29 - DNA, 1389 bp, Homo sapiens
atgggggcgagcttcctgcagctgcagagcatcaaagacgcctgctgcacattccttcgagaacggcttcacccaaaaaactgcctgggtgtgcgccagtttgctgagacaatgatgtgtgctgtgctgtacgacgctgccaacagcttcatccaccagcactttgtggaggtgtccatgtcagaagagttcctggccctgcccttggaagacgtgcttgagctggtgtctcgggatgagctgaatgtcaaatctgaggagcaggtctttgaagctgcattggcctgggtcagatacgaccgggagcagaggggtccctacctgcctgagctgctgtccaatatccgcctgcccctctgtcggccccagttcctttcagacagagtacagcaggatgacctggtgcgttgctgccacaaatgcagggacctggtagacgaagcaaaggactaccacctcatgccagagcgccggccccacctgccagctttcagaacccggccacgctgctgcacatccatcgctggacttatctacgctgtagggggcctcaactcagcaggtgattccctgaatgtggtggaagtgttcgaccccattgccaattgctgggagagatgccgtcccatgacaacagcccgcagccgcgttggcgtggctgtggtgaacgggcttctctatgccatcggaggatatgacggccagctacggctgagcactgtggaggcctacaacccggagacagacacatggaccagagtggggagcatgaatagcaagagaagtgccatggggacagtcgtgctggatgggcagatctacgtctgtgggggctacgatggcaactcttccctcagctccgtggagacctactcacctgagacggacaaatggacagtggtgacctcgatgagctcgaatcgcagtgctgctggggttacagtctttgagggcaggatatatgtgtcaggcggccatgatggtttgcagatcttcagcagtgtggaacactacaaccaccacacagccacctggcaccctgcagctggcatgctcaacaagcgctgccggcacggagccgcctccctggggagcaagatgtttgtctgcgggggctacgatggctctggcttcctcagcattgccgagatgtacagctctgtggcagaccagtggtgcctgattgtccccatgcacacgcgcaggagccgggtctccctggtggccagctgtgggcgcctctacgctgttgggggctacgacggacagtcaaacctaagctcagtggagatgtatgacccagagacagactgctggacattcatggcccccatggcgtgccatgagggaggggtcggtgtgggctgcatccctctcctcaccatctaa

SEQ ID NO: 30 - protein, 462 aa, Homo sapiens
MGASFLQLQSIKDACCTFLRERLHPKNCLGVRQFAETMMCAVLYDAANSFIHQHFVEVSMSEEFLALPLEDVLELVSRDELNVKSEEQVFEAALAWVRYDREQRGPYLPELLSNIRLPLCRPQFLSDRVQQDDLVRCCHKCRDLVDEAKDYHLMPERRPHLPAFRTRPRCCTSIAGLIYAVGGLNSAGDSLNVVEVFDPIANCWERCRPMTTARSRVGVAVVNGLLYAIGGYDGQLRLSTVEAYNPETDTWTRVGSMNSKRSAMGTVVLDGQIYVCGGYDGNSSLSSVETYSPETDKWTVVTSMSSNRSAAGVTVFEGRIYVSGGHDGLQIFSSVEHYNHHTATWHPAAGMLNKRCRHGAASLGSKMFVCGGYDGSGFLSIAEMYSSVADQWCLIVPMHTRRSRVSLVASCGRLYAVGGYDGQSNLSSVEMYDPETDCWTFMAPMACHEGGVGVGCIPLLTI

SEQ ID NO: 31 - DNA, 4612 bp, Homo sapiens
ccaactgaattttcagatgagatgagaaggtcatgcttttccacctttgagctcccactttgaccagctctgccagtcctgagccagaaggtcaacagttaaaaagaagagattggggaccacaaattcagtgcccaccggattgtcttagcagcctcgatcccgtatttccatgctatgtttacaaatgacatgatggagtgcaagcaggatgagattgtaatgcaaggaatggacccaagtgccctggaggctctgatcaactttgcctacaacggcaaccttgccattgaccagcaaaatgtccagtcattgctgatgggggcgagcttcctgcagctgcagagcatcaaagacgcctgctgcacattccttcgagaacggcttcacccaaaaaactgcctgggtgtgcgccagtttgctgagacaatgatgtgtgctgtgctgtacgacgctgccaacagcttcatccaccagcactttgtggaggtgtccatgtcagaagagttcctggccctgcccttggaagacgtgcttgagctggtgtctcgggatgagctgaatgtcaaatctgaggagcaggtctttgaagctgcattggcctgggtcagatacgaccgggagcagaggggtccctacctgcctgagctgctgtccaatatccgcctgcccctctgtcggccccagttcctttcagacagagtacagcaggatgacctggtgcgttgctgccacaaatgcagggacctggtagacgaagcaaaggactaccacctcatgccagagcgccggccccacctgccagctttcagaacccggccacgctgctgcacatccatcgctggacttatctacgctgtagggggcctcaactcagcagcaaatttttatgcaggtgattccctgaatgtggtggaagtgttcgaccccattgccaattgctgggagagatgccgtcccatgacaacagcccgcagccgcgttggcgtggctgtggtgaacgggcttctctatgccatcggaggatatgacggccagctacggctgagcactgtggaggcctacaacccggagacagacacatggaccagagtggggagcatgaatagcaagagaagctctgtctgtttcagtgccatggggacagtcgtgctggatgggcagatctacgtctgtgggggctacgatggcaactcttccctcagctccgtggagacctactcacctgagacggacaaatggacagtggtgacctcgatgagctcgaatcgcagtgctgctggggttacagtctttgagggcaggatatatgtgtcaggcggccatgatggtttgcagatcttcagcagtgtggaacactacaaccaccacacagccacctggcaccctgcagctggcatgctcaacaagcgctgccggcacggagccgcctccctggggagcaagatgtttgtctgcgggggctacgatggctctggcttcctcagcattgccgagatgtacagctctgtggcagaccagtggtgcctgattgtccccatgcacacgcgcaggagccgggtctccctggtggccagctgtgggcgcctctacgctgttgggggctacgacggacagtcaaacctaagctcagtggagatgtatgacccagagacagactgctggacattcatggcccccatggcgtgccatgagggaggggtcggtgtgggctgcatccctctcctcaccatctaaggcagaggatgggatgtggtggggcagggatctggtacagacataggcgcttccttccaggaacagtccctcaggagaggcagtggaccagaagagatggcgaaacgtgagctcgccggaggtacagtttttccaggtgcttaagccctcccccactgtgccacccttgtgaccttcaggcttgggtcatcaagatgcacagcatggaacacaagctcctctggatcctgcagctggtgacatggaactgttttctggtccacatgaacacaggctccatccaggcccagctcctacccaccgcctctctgtgggccagctgttcacagaaggccttccatctgatgctccccatcgcctgcttgctctccagccgagtctggccaatttgccatggggaggctgcagtgtccaagcctgctggaaactgggatgtagctggggacgaaaggacagacccaagcgttctccctgcctgagatggtgtggccacagcagtggaaggctgcacacaggcacattccttcttccacagtggggcaccaaggattctgtcctcattgctgggtaagcagggagaagagaagttttccccatgtctaattttgggatttcagtgaggccttttgatctgtccaggagaacagaagggaaaaaaagatacttgaaagaaactgaaggaaatttaaacaaagaaacacttgaaagaaactggaaagaaaaataatttttttatgtgaacaaattttgcaagaagaaaaaagcataaaagacactaacggcaaatctatgtttaaatggaaaatcgtctaactggagaagggcggtatccaccccacattcggatcccagggtcctgaggcctcgcattgagctgggggttccctctgagccccagtgtgtgtggaatcagtgcactcttgactgggcctgtagtaaggtgctcatggggtttgtcttctcacccaccatcagaggacttttaaaatcataggcgtagagagttaggctatctgctgaattactgccactcttcttggtgggggctcctagctgtggctgggggctccaggcgcccctgtgattacctcctactgccaccatggcgctcattcagattccccactctcactaacattgcttccttttttgaccagcaggaaacagcaggtctggccagattctcacttgcccatcaatctcgttcttggatgatttccctcattgtgatgcttctggggcacgttgaccatatgcacctctagaacctaaccagggcttccttctaccagctgtgggcgggcttggtctggtaaccttgtctgctctgccattccactgctcctccatccactcgccaatcccaagagtctggcctccctccagccctgggcagactgaccagcaaggtggacctttacattcaagcacagctggcttttatgacataaagaactaaaggccgaaagaatctcttgctgctgcaaagaacagattttatatttcttcctctaatcttggcaaatgacctttaccttttggaaagatttcatattgcttcctcctccctggataggacctaatgtagcacagcgggactcaaagaggaggacattttctcttgccagtgcactgggcagtggggctgtccttcaactgctgctgccaaaattggttttctaaaattcttccagtagagactaaaagaagattcaattcctgtaacccaagactgagtcttagggctccagtctccacctgcttggtttcctatcctttgctgcctgcctggggtggcctggaagcctgttcagaaaggcacaatgtggagcctggggtgtctcccccaccccaggaccgtcaggtttaccagtgtgtgcaatcgccatgtattcagagggaagtacctttgttacctacaacttaggagctaggcctctgctacaagcacttgaaaatgatatttttatttttaacgtctcaacaatctgatatcggatgtcgtttaacctgggctcgtggtagggctccagcatttctccctccttcctggtttgcctgtaggggtagactcggaaggtgggtggggtgtgcatttcctgttaggagtgtatcagtgcttgtcttattataagcccctttcttttgtgaatttgaagtagcaccaacaagcctggattgtgaaggtattaagaatcggtctgtgggctactgagtgggtccttaggatactggcccagattttgccactgggtatggcagatcattttctaccatggcctgctgctcttgtagtggacttcctgagtccaatcccacctcctggtgtagaatttacactgctgcacctgaggtcgatgtttcaaagtaagatcaagccagtgttttgatctgggctctgagcacaagtcaggaaacaccaacatattcacactctcccagtaggttcctcagtccgatggtgaatggctattcgtaaatggctggtctggctctttggtgttggagcctttccaatagccccatgaaaagaagcatcacccaaggatattgtaaaaaggatgtaacaaggagatagggtagacattgtactcagtgggccttggggcctagcccagctctgagcagaggactgtggcattcactgtccttgagtgtttcaccttcttggataacacacgggccttctcttctggatttcatcagagattacagccagatgggggctgaagaccatcctcttgaccacagaggtgtgactgtgggaattcctcccaatttatggtttcccagaaaatcttagttccttttatttatagaatgcatgtcttttgtgttaagaaaccaaagagaaataaagagaacactcctaata

SEQ ID NO: 32 - DNA, 1419 bp, Homo sapiens; identical to SEQ ID NO: 23

SEQ ID NO: 33 - protein, 519 aa, Homo sapiens
MFTNDMMECKQDEIVMQGMDPSALEALINFAYNGNLAIDQQNVQSLLMGASFLQLQSIKDACCTFLRERLHPKNCLGVRQFAETMMCAVLYDAANSFIHQHFVEVSMSEEFLALPLEDVLELVSRDELNVKSEEQVFEAALAWVRYDREQRGPYLPELLSNIRLPLCRPQFLSDRVQQDDLVRCCHKCRDLVDEAKDYHLMPERRPHLPAFRTRPRCCTSIAGLIYAVGGLNSAANFYAGDSLNVVEVFDPIANCWERCRPMTTARSRVGVAVVNGLLYAIGGYDGQLRLSTVEAYNPETDTWTRVGSMNSKRSSVCFSAMGTVVLDGQIYVCGGYDGNSSLSSVETYSPETDKWTVVTSMSSNRSAAGVTVFEGRIYVSGGHDGLQIFSSVEHYNHHTATWHPAAGMLNKRCRHGAASLGSKMFVCGGYDGSGFLSIAEMYSSVADQWCLIVPMHTRRSRVSLVASCGRLYAVGGYDGQSNLSSVEMYDPETDCWTFMAPMACHEGGVGVGCIPLLTI

SEQ ID NO: 34 - DNA, 1398 bp, Mus musculus
ttcccctggctccagccggcgcaagcagcggcggcggtggcagcgggcgaggatctgcggccccgcgaggccatgaaggtgaagaaaggcggcggcgggaccgggtcgggggcggagcccgttccaggggcctcgaaccggagcgcggagcccacgcgggagcctggggcggaagctgagtccgggtccgagtcggagccggagccaggcccggggcccaggctggggccgctgcagggcaagcagcccatcgggccggaggatgtgctggggctgcagcggatcacgggtgactacctgtgctcccctgaggaaaatatctacaagattgacttcgtcaggttcaagatccgtgacatggactcagggactgtcctttttgaaatcaagaagccccctgtttcggaacggttgcccatcaaccggcgggacctggaccccaatgcagggcgctttgttcgctaccagttcacacctgccttcctccgcctaaggcaggtgggagccacggtggagttcacagtgggagacaagccggtcaacaacttccgcatgatcgagaggcactactttcgaaaccagctcctcaaaagcttcgacttccactttggcttctgcatccccagcagcaagaacacctgtgagcacatctatgacttccctcctctctccgaggagctaattctgaagtccctacagggtctggctcagggtcctgacctttgccctggatgggcctctcttgcagtcagtgagatgattcgtcacccgtatgagacccagtctgacagcttctacttcgtggatgaccggctggtgatgcataacaaagcagactattcctacagtgggacaccctgacccctaatgctgcccctgaggctctggcctagaccctgtgctgtaacctctccgacatcatctccacttggggatggatccggtggctctggaccctgagtcagtctcgagaggaaaggtgtccagcatccctaggcaaacctctggagctagtgggaggggcagcagggggaggctggctgtccccatgttcaggaaggcctcctgcaagaggaggactcctggatgcctcgctaggtccactgggcctgagtttcagagtagtgcccccttcttgaccgtgactagatcaggttagggaccatttcctgtcccttgcccaccacctccaggctatttatagttgtcggttcacagacaaagatccacagtgggtaccctgctctgagccctggcctcctccatcaggggccaagaaactacccgaggtgtgagaggggcgggtccagatcgcagcctgtaagacctggacaaactgtatatagttttcaataaaccttttctgttcttgggtgcggccaaaaaaaaaaaaaaaaa

SEQ ID NO: 35 - DNA, 789 bp, Mus musculus
atgaaggtgaagaaaggcggcggcgggaccgggtcgggggcggagcccgttccaggggcctcgaaccggagcgcggagcccacgcgggagcctggggcggaagctgagtccgggtccgagtcggagccggagccaggcccggggcccaggctggggccgctgcagggcaagcagcccatcgggccggaggatgtgctggggctgcagcggatcacgggtgactacctgtgctcccctgaggaaaatatctacaagattgacttcgtcaggttcaagatccgtgacatggactcagggactgtcctttttgaaatcaagaagccccctgtttcggaacggttgcccatcaaccggcgggacctggaccccaatgcagggcgctttgttcgctaccagttcacacctgccttcctccgcctaaggcaggtgggagccacggtggagttcacagtgggagacaagccggtcaacaacttccgcatgatcgagaggcactactttcgaaaccagctcctcaaaagcttcgacttccactttggcttctgcatccccagcagcaagaacacctgtgagcacatctatgacttccctcctctctccgaggagctaattctgaagtccctacagggtctggctcagggtcctgacctttgccctggatgggcctctcttgcagtcagtgagatgattcgtcacccgtatgagacccagtctgacagcttctacttcgtggatgaccggctggtgatgcataacaaagcagactattcctacagtgggacaccctga

SEQ ID NO: 36 - protein, 262 aa, Mus musculus
MKVKKGGGGTGSGAEPVPGASNRSAEPTREPGAEAESGSESEPEPGPGPRLGPLQGKQPIGPEDVLGLQRITGDYLCSPEENIYKIDFVRFKIRDMDSGTVLFEIKKPPVSERLPINRRDLDPNAGRFVRYQFTPAFLRLRQVGATVEFTVGDKPVNNFRMIERHYFRNQLLKSFDFHFGFCIPSSKNTCEHIYDFPPLSEELILKSLQGLAQGPDLCPGWASLAVSEMIRHPYETQSDSFYFVDDRLVMHNKADYSYSGTP

SEQ ID NO: 37 - DNA, 1156 bp, Mus musculus
gtcctctcaagaccagccttgcctgatgaatgtagatgtcatgccacaggactacctgtgctcccctgaggaaaatatctacaagattgacttcgtcaggttcaagatccgtgacatggactcagggactgtcctttttgaaatcaagaagccccctgtttcggaacggttgcccatcaaccggcgggacctggaccccaatgcagggcgctttgttcgctaccagttcacacctgccttcctccgcctaaggcaggtgggagccacggtggagttcacagtgggagacaagccggtcaacaacttccgcatgatcgagaggcactactttcgaaaccagctcctcaaaagcttcgacttccactttggcttctgcatccccagcagcaagaacacctgtgagcacatctatgacttccctcctctctccgaggagctaattctgaagtccctacagggtctggctcagggtcctgacctttgccctggatgggcctctcttgcagtcagtgagatgattcgtcacccgtatgagacccagtctgacagcttctacttcgtggatgaccggctggtgatgcataacaaagcagactattcctacagtgggacaccctgacccctaatgctgcccctgaggctctggcctagaccctgtgctgtaacctctccgacatcatctccacttggggatggatccggtggctctggaccctgagtcagtctcgagaggaaaggtgtccagcatccctaggcaaacctctggagctagtgggaggggcagcagggggaggctggctgtccccatgttcaggaaggcctcctgcaagaggaggactcctggatgcctcgctaggtccactgggcctgagtttcagagtagtgcccccttcttgaccgtgactagatcaggttagggaccatttcctgtcccttgcccaccacctccaggctatttatagttgtcggttcacagacaaagatccacagtgggtaccctgctctgagccctggcctcctccatcaggggccaagaaactacccgaggtgtgagaggggcgggtccagatcgcagcctgtaagacctggacaaactgtatatagttttcaataaaccttttctgttcttgggtgcggccaaaaaaaaaaaaaaaaa

SEQ ID NO: 38 - DNA, 594 bp, Mus musculus
atgaatgtagatgtcatgccacaggactacctgtgctcccctgaggaaaatatctacaagattgacttcgtcaggttcaagatccgtgacatggactcagggactgtcctttttgaaatcaagaagccccctgtttcggaacggttgcccatcaaccggcgggacctggaccccaatgcagggcgctttgttcgctaccagttcacacctgccttcctccgcctaaggcaggtgggagccacggtggagttcacagtgggagacaagccggtcaacaacttccgcatgatcgagaggcactactttcgaaaccagctcctcaaaagcttcgacttccactttggcttctgcatccccagcagcaagaacacctgtgagcacatctatgacttccctcctctctccgaggagctaattctgaagtccctacagggtctggctcagggtcctgacctttgccctggatgggcctctcttgcagtcagtgagatgattcgtcacccgtatgagacccagtctgacagcttctacttcgtggatgaccggctggtgatgcataacaaagcagactattcctacagtgggacaccctga

SEQ ID NO: 39 - protein, 197 aa, Mus musculus
MNVDVMPQDYLCSPEENIYKIDFVRFKIRDMDSGTVLFEIKKPPVSERLPINRRDLDPNAGRFVRYQFTPAFLRLRQVGATVEFTVGDKPVNNFRMIERHYFRNQLLKSFDFHFGFCIPSSKNTCEHIYDFPPLSEELILKSLQGLAQGPDLCPGWASLAVSEMIRHPYETQSDSFYFVDDRLVMHNKADYSYSGTP

SEQ ID NO: 40 - DNA, 1090 bp, Mus musculus
gtcctctcaagaccagccttgcctgatgaatgtagatgtcatgccacaggactacctgtgctcccctgaggaaaatatctacaagattgacttcgtcaggttcaagatccgtgacatggactcagggactgtcctttttgaaatcaagaagccccctgtttcggaacggttgcccatcaaccggcgggacctggaccccaatgcagggcgctttgttcgctaccagttcacacctgccttcctccgcctaaggcaggtgggagccacggtggagttcacagtgggagacaagccggtcaacaacttccgcatgatcgagaggcactactttcgaaaccagctcctcaaaagcttcgacttccactttggcttctgcatccccagcagcaagaacacctgtgagcacatctatgacttccctcctctctccgaggagctaatcagtgagatgattcgtcacccgtatgagacccagtctgacagcttctacttcgtggatgaccggctggtgatgcataacaaagcagactattcctacagtgggacaccctgacccctaatgctgcccctgaggctctggcctagaccctgtgctgtaacctctccgacatcatctccacttggggatggatccggtggctctggaccctgagtcagtctcgagaggaaaggtgtccagcatccctaggcaaacctctggagctagtgggaggggcagcagggggaggctggctgtccccatgttcaggaaggcctcctgcaagaggaggactcctggatgcctcgctaggtccactgggcctgagtttcagagtagtgcccccttcttgaccgtgactagatcaggttagggaccatttcctgtcccttgcccaccacctccaggctatttatagttgtcggttcacagacaaagatccacagtgggtaccctgctctgagccctggcctcctccatcaggggccaagaaactacccgaggtgtgagaggggcgggtccagatcgcagcctgtaagacctggacaaactgtatatagttttcaataaaccttttctgttcttgggtgcggccaaaaaaaaaaaaaaaaa

SEQ ID NO: 41 - DNA, 528 bp, Mus musculus
atgaatgtagatgtcatgccacaggactacctgtgctcccctgaggaaaatatctacaagattgacttcgtcaggttcaagatccgtgacatggactcagggactgtcctttttgaaatcaagaagccccctgtttcggaacggttgcccatcaaccggcgggacctggaccccaatgcagggcgctttgttcgctaccagttcacacctgccttcctccgcctaaggcaggtgggagccacggtggagttcacagtgggagacaagccggtcaacaacttccgcatgatcgagaggcactactttcgaaaccagctcctcaaaagcttcgacttccactttggcttctgcatccccagcagcaagaacacctgtgagcacatctatgacttccctcctctctccgaggagctaatcagtgagatgattcgtcacccgtatgagacccagtctgacagcttctacttcgtggatgaccggctggtgatgcataacaaagcagactattcctacagtgggacaccctga

SEQ ID NO: 42 - protein, 175 aa, Mus musculus
MNVDVMPQDYLCSPEENIYKIDFVRFKIRDMDSGTVLFEIKKPPVSERLPINRRDLDPNAGRFVRYQFTPAFLRLRQVGATVEFTVGDKPVNNFRMIERHYFRNQLLKSFDFHFGFCIPSSKNTCEHIYDFPPLSEELISEMIRHPYETQSDSFYFVDDRLVMHNKADYSYSGTP

SEQ ID NO: 43 - DNA, 1139 bp, Mus musculus
ctttttcttggctgaggagaggaagtggctgccttcctaggcagcccctgatcctcgctccttgtaagggcagagaggcccacaagttgagtttgcagtactacctgtgctcccctgaggaaaatatctacaagattgacttcgtcaggttcaagatccgtgacatggactcagggactgtcctttttgaaatcaagaagccccctgtttcggaacggttgcccatcaaccggcgggacctggaccccaatgcagggcgctttgttcgctaccagttcacacctgccttcctccgcctaaggcaggtgggagccacggtggagttcacagtgggagacaagccggtcaacaacttccgcatgatcgagaggcactactttcgaaaccagctcctcaaaagcttcgacttccactttggcttctgcatccccagcagcaagaacacctgtgagcacatctatgacttccctcctctctccgaggagctaatcagtgagatgattcgtcacccgtatgagacccagtctgacagcttctacttcgtggatgaccggctggtgatgcataacaaagcagactattcctacagtgggacaccctgacccctaatgctgcccctgaggctctggcctagaccctgtgctgtaacctctccgacatcatctccacttggggatggatccggtggctctggaccctgagtcagtctcgagaggaaaggtgtccagcatccctaggcaaacctctggagctagtgggaggggcagcagggggaggctggctgtccccatgttcaggaaggcctcctgcaagaggaggactcctggatgcctcgctaggtccactgggcctgagtttcagagtagtgcccccttcttgaccgtgactagatcaggttagggaccatttcctgtcccttgcccaccacctccaggctatttatagttgtcggttcacagacaaagatccacagtgggtaccctgctctgagccctggcctcctccatcaggggccaagaaactacccgaggtgtgagaggggcgggtccagatcgcagcctgtaagacctggacaaactgtatatagttttcaataaaccttttctgttcttgggtgcggccaaaaaaaaaaaaaaaaa

SEQ ID NO: 44 - DNA, 438 bp, Mus musculus
atggactcagggactgtcctttttgaaatcaagaagccccctgtttcggaacggttgcccatcaaccggcgggacctggaccccaatgcagggcgctttgttcgctaccagttcacacctgccttcctccgcctaaggcaggtgggagccacggtggagttcacagtgggagacaagccggtcaacaacttccgcatgatcgagaggcactactttcgaaaccagctcctcaaaagcttcgacttccactttggcttctgcatccccagcagcaagaacacctgtgagcacatctatgacttccctcctctctccgaggagctaatcagtgagatgattcgtcacccgtatgagacccagtctgacagcttctacttcgtggatgaccggctggtgatgcataacaaagcagactattcctacagtgggacaccctga

SEQ ID NO: 45 - protein, 145 aa, Mus musculus
MDSGTVLFEIKKPPVSERLPINRRDLDPNAGRFVRYQFTPAFLRLRQVGATVEFTVGDKPVNNFRMIERHYFRNQLLKSFDFHFGFCIPSSKNTCEHIYDFPPLSEELISEMIRHPYETQSDSFYFVDDRLVMHNKADYSYSGTP

SEQ ID NO: 46 - DNA, 1332 bp, Mus musculus
ttcccctggctccagccggcgcaagcagcggcggcggtggcagcgggcgaggatctgcggccccgcgaggccatgaaggtgaagaaaggcggcggcgggaccgggtcgggggcggagcccgttccaggggcctcgaaccggagcgcggagcccacgcgggagcctggggcggaagctgagtccgggtccgagtcggagccggagccaggcccggggcccaggctggggccgctgcagggcaagcagcccatcgggccggaggatgtgctggggctgcagcggatcacgggtgactacctgtgctcccctgaggaaaatatctacaagattgacttcgtcaggttcaagatccgtgacatggactcagggactgtcctttttgaaatcaagaagccccctgtttcggaacggttgcccatcaaccggcgggacctggaccccaatgcagggcgctttgttcgctaccagttcacacctgccttcctccgcctaaggcaggtgggagccacggtggagttcacagtgggagacaagccggtcaacaacttccgcatgatcgagaggcactactttcgaaaccagctcctcaaaagcttcgacttccactttggcttctgcatccccagcagcaagaacacctgtgagcacatctatgacttccctcctctctccgaggagctaatcagtgagatgattcgtcacccgtatgagacccagtctgacagcttctacttcgtggatgaccggctggtgatgcataacaaagcagactattcctacagtgggacaccctgacccctaatgctgcccctgaggctctggcctagaccctgtgctgtaacctctccgacatcatctccacttggggatggatccggtggctctggaccctgagtcagtctcgagaggaaaggtgtccagcatccctaggcaaacctctggagctagtgggaggggcagcagggggaggctggctgtccccatgttcaggaaggcctcctgcaagaggaggactcctggatgcctcgctaggtccactgggcctgagtttcagagtagtgcccccttcttgaccgtgactagatcaggttagggaccatttcctgtcccttgcccaccacctccaggctatttatagttgtcggttcacagacaaagatccacagtgggtaccctgctctgagccctggcctcctccatcaggggccaagaaactacccgaggtgtgagaggggcgggtccagatcgcagcctgtaagacctggacaaactgtatatagttttcaataaaccttttctgttcttgggtgcggccaaaaaaaaaaaaaaaaa

SEQ ID NO: 47 - DNA, 723 bp, Mus musculus
atgaaggtgaagaaaggcggcggcgggaccgggtcgggggcggagcccgttccaggggcctcgaaccggagcgcggagcccacgcgggagcctggggcggaagctgagtccgggtccgagtcggagccggagccaggcccggggcccaggctggggccgctgcagggcaagcagcccatcgggccggaggatgtgctggggctgcagcggatcacgggtgactacctgtgctcccctgaggaaaatatctacaagattgacttcgtcaggttcaagatccgtgacatggactcagggactgtcctttttgaaatcaagaagccccctgtttcggaacggttgcccatcaaccggcgggacctggaccccaatgcagggcgctttgttcgctaccagttcacacctgccttcctccgcctaaggcaggtgggagccacggtggagttcacagtgggagacaagccggtcaacaacttccgcatgatcgagaggcactactttcgaaaccagctcctcaaaagcttcgacttccactttggcttctgcatccccagcagcaagaacacctgtgagcacatctatgacttccctcctctctccgaggagctaatcagtgagatgattcgtcacccgtatgagacccagtctgacagcttctacttcgtggatgaccggctggtgatgcataacaaagcagactattcctacagtgggacaccctga

SEQ ID NO: 48 - protein, 240 aa, Mus musculus
MKVKKGGGGTGSGAEPVPGASNRSAEPTREPGAEAESGSESEPEPGPGPRLGPLQGKQPIGPEDVLGLQRITGDYLCSPEENIYKIDFVRFKIRDMDSGTVLFEIKKPPVSERLPINRRDLDPNAGRFVRYQFTPAFLRLRQVGATVEFTVGDKPVNNFRMIERHYFRNQLLKSFDFHFGFCIPSSKNTCEHIYDFPPLSEELISEMIRHPYETQSDSFYFVDDRLVMHNKADYSYSGTP

SEQ ID NO: 49 - DNA, 1398 bp, Homo sapiens
cccacttcccccggctccagccggcgcaggcagcggcggcagcagcaggcgagcctcggccccgcaaggccatgaaggtgaagaagggcggcggtggggccgggacggcgacggagtccgctccggggccctcgggccagagcgtggcccccataccacagccgcctgcggaatccgaatctgggtccgagtcggagccggacgcaggcccagggcccaggccggggccgctgcagaggaagcagccgatcgggccggaggacgtgctggggctgcagcggatcaccggtgactacctctgctcccctgaggagaatatctacaagatcgactttgtcaggtttaagattcgggacatggactcaggcactgtcctctttgaaatcaagaagcccccagtctcagaacggttgcccatcaaccggcgggacctggaccccaatgctgggcgctttgtccgctaccagttcacgcctgccttcctccgcctgaggcaggtgggagccacggtggagttcacagtgggagacaagcctgtcaacaacttccgcatgatcgagaggcactacttccgcaaccagctactcaaaagcttcgacttccactttggcttctgcatccccagcagcaagaacacctgcgagcacatttacgacttcccccctctctccgaggagctgatcagcgagatgatccgccacccgtatgagacccagtctgacagcttctacttcgtggatgaccggctggtgatgcacaataaagcagactattcctacagcgggacaccctgaccccacggctgccctgaccccaggaggctccagttctgggctgggagctgtgacctccccaacgctcacccctcaaccccaagtcctctgcttggggagttctccaggagctccggaccctgagtcaatgttgggaggaagggtacctggtgtccccagtcaagcccatgaagcccatgcggcctgctacatggggtggggtcgtagggaggctgtttgcctccacgtctaggaaggcctgtgagaggagcagtcaggacttccggacaacttagctgggccctacttgggcccaagtttcagaatagtgttcccctatcaaggctgtgactagatcaggcagggatccattccctgtcccctgcccactaccttcaggccatttagagttgtaaatttacaaagatccacggtgggctccagctgccaagccacccaagggagtctgggccctaggcctagccccatccctccccatgaggggccaagacactgcctaaggtgtgggagggactggctgagattgcagcccatggtaggagctggaccaactgtatatagttttcaataaactttttccttttctgttcaaaaaaaaaaaaaa

SEQ ID NO: 50 - DNA, 723 bp, Homo sapiens
atgaaggtgaagaagggcggcggtggggccgggacggcgacggagtccgctccggggccctcgggccagagcgtggcccccataccacagccgcctgcggaatccgaatctgggtccgagtcggagccggacgcaggcccagggcccaggccggggccgctgcagaggaagcagccgatcgggccggaggacgtgctggggctgcagcggatcaccggtgactacctctgctcccctgaggagaatatctacaagatcgactttgtcaggtttaagattcgggacatggactcaggcactgtcctctttgaaatcaagaagcccccagtctcagaacggttgcccatcaaccggcgggacctggaccccaatgctgggcgctttgtccgctaccagttcacgcctgccttcctccgcctgaggcaggtgggagccacggtggagttcacagtgggagacaagcctgtcaacaacttccgcatgatcgagaggcactacttccgcaaccagctactcaaaagcttcgacttccactttggcttctgcatccccagcagcaagaacacctgcgagcacatttacgacttcccccctctctccgaggagctgatcagcgagatgatccgccacccgtatgagacccagtctgacagcttctacttcgtggatgaccggctggtgatgcacaataaagcagactattcctacagcgggacaccctga

SEQ ID NO: 51 - protein, 240 aa, Homo sapiens
MKVKKGGGGAGTATESAPGPSGQSVAPIPQPPAESESGSESEPDAGPGPRPGPLQRKQPIGPEDVLGLQRITGDYLCSPEENIYKIDFVRFKIRDMDSGTVLFEIKKPPVSERLPINRRDLDPNAGRFVRYQFTPAFLRLRQVGATVEFTVGDKPVNNFRMIERHYFRNQLLKSFDFHFGFCIPSSKNTCEHIYDFPPLSEELISEMIRHPYETQSDSFYFVDDRLVMHNKADYSYSGTP

SEQ ID NO: 52 - DNA, 1665 bp, Homo sapiens
cccacttcccccggctccagccggcgcaggcagcggcggcagcagcaggcgagcctcggccccgcaaggccatgaaggtgaagaagggcggcggtggggccgggacggcgacggagtccgctccggggccctcgggccagagcgtggcccccataccacagccgcctgcggaatccgaatctgggtccgagtcggagccggacgcaggcccagggcccaggccggggccgctgcagaggaagcagccgatcgggccggaggacgtgctggggctgcagcggatcaccggtgactacctctgctcccctgaggagaatatctacaagatcgactttgtcaggtttaagattcgggacatggactcaggcactgtcctctttgaaatcaagaagcccccagtctcagaacggttgcccatcaaccggcgggacctggaccccaatgctgggcgctttgtccgctaccagttcacgcctgccttcctccgcctgaggcaggtgggagccacggtggagttcacagtgggagacaagcctgtcaacaacttccgcatgatcgagaggcactacttccgcaaccagctactcaaaagcttcgacttccactttggcttctgcatccccagcagcaagaacacctgcgagcacatttacgacttcccccctctctccgaggagctgagtgcgcgggcagggtcttctgggagtggggaagtgggggcgtctagagactgagctgcgggagggagagggacttgtgggtctgatcccatttctccccaccctggggctcttctgtgtctgccaccattcccatatcatccgtagagaaagaggctggggatatttcaggctgtttggctgtccctgtaccccagtcctgaagcccctgcagtggcgggactcaagctcctgacctttgcccggcctggctgggcctctcttgcagtcagcgagatgatccgccacccgtatgagacccagtctgacagcttctacttcgtggatgaccggctggtgatgcacaataaagcagactattcctacagcgggacaccctgaccccacggctgccctgaccccaggaggctccagttctgggctgggagctgtgacctccccaacgctcacccctcaaccccaagtcctctgcttggggagttctccaggagctccggaccctgagtcaatgttgggaggaagggtacctggtgtccccagtcaagcccatgaagcccatgcggcctgctacatggggtggggtcgtagggaggctgtttgcctccacgtctaggaaggcctgtgagaggagcagtcaggacttccggacaacttagctgggccctacttgggcccaagtttcagaatagtgttcccctatcaaggctgtgactagatcaggcagggatccattccctgtcccctgcccactaccttcaggccatttagagttgtaaatttacaaagatccacggtgggctccagctgccaagccacccaagggagtctgggccctaggcctagccccatccctccccatgaggggccaagacactgcctaaggtgtgggagggactggctgagattgcagcccatggtaggagctggaccaactgtatatagttttcaataaactttttccttttctgttcaaaaaaaaaaaaaa

SEQ ID NO: 53 - DNA, 663 bp, Homo sapiens
atgaaggtgaagaagggcggcggtggggccgggacggcgacggagtccgctccggggccctcgggccagagcgtggcccccataccacagccgcctgcggaatccgaatctgggtccgagtcggagccggacgcaggcccagggcccaggccggggccgctgcagaggaagcagccgatcgggccggaggacgtgctggggctgcagcggatcaccggtgactacctctgctcccctgaggagaatatctacaagatcgactttgtcaggtttaagattcgggacatggactcaggcactgtcctctttgaaatcaagaagcccccagtctcagaacggttgcccatcaaccggcgggacctggaccccaatgctgggcgctttgtccgctaccagttcacgcctgccttcctccgcctgaggcaggtgggagccacggtggagttcacagtgggagacaagcctgtcaacaacttccgcatgatcgagaggcactacttccgcaaccagctactcaaaagcttcgacttccactttggcttctgcatccccagcagcaagaacacctgcgagcacatttacgacttcccccctctctccgaggagctgagtgcgcgggcagggtcttctgggagtggggaagtgggggcgtctagagactga

SEQ ID NO: 54 - protein, 220 aa, Homo sapiens
MKVKKGGGGAGTATESAPGPSGQSVAPIPQPPAESESGSESEPDAGPGPRPGPLQRKQPIGPEDVLGLQRITGDYLCSPEENIYKIDFVRFKIRDMDSGTVLFEIKKPPVSERLPINRRDLDPNAGRFVRYQFTPAFLRLRQVGATVEFTVGDKPVNNFRMIERHYFRNQLLKSFDFHFGFCIPSSKNTCEHIYDFPPLSEELSARAGSSGSGEVGASRD

SEQ ID NO: 55 - DNA, 1461 bp, Homo sapiens
ctggggccccggccgggggcggggctgcggatgctcccacttcccccggctccagccggcgcaggcagcggcggcagcagcaggcgagcctcggccccgcaaggccatgaaggtgaagaagggcggcggtggggccgggacggcgacggagtccgctccggggccctcgggccagagcgtggcccccataccacagccgcctgcggaatccgaatctgggtccgagtcggagccggacgcaggcccagggcccaggccggggccgctgcagaggaagcagccgatcgggccggaggacgtgctggggctgcagcggatcaccggtggggcccgtccccttttcccagcgtggagactacctctgctcccctgaggagaatatctacaagatcgactttgtcaggtttaagattcgggacatggactcaggcactgtcctctttgaaatcaagaagcccccagtctcagaacggttgcccatcaaccggcgggacctggaccccaatgctgggcgctttgtccgctaccagttcacgcctgccttcctccgcctgaggcaggtgggagccacggtggagttcacagtgggagacaagcctgtcaacaacttccgcatgatcgagaggcactacttccgcaaccagctactcaaaagcttcgacttccactttggcttctgcatccccagcagcaagaacacctgcgagcacatttacgacttcccccctctctccgaggagctgatcagcgagatgatccgccacccgtatgagacccagtctgacagcttctacttcgtggatgaccggctggtgatgcacaataaagcagactattcctacagcgggacaccctgaccccacggctgccctgaccccaggaggctccagttctgggctgggagctgtgacctccccaacgctcacccctcaaccccaagtcctctgcttggggagttctccaggagctccggaccctgagtcaatgttgggaggaagggtacctggtgtccccagtcaagcccatgaagcccatgcggcctgctacatggggtggggtcgtagggaggctgtttgcctccacgtctaggaaggcctgtgagaggagcagtcaggacttccggacaacttagctgggccctacttgggcccaagtttcagaatagtgttcccctatcaaggctgtgactagatcaggcagggatccattccctgtcccctgcccactaccttcaggccatttagagttgtaaatttacaaagatccacggtgggctccagctgccaagccacccaagggagtctgggccctaggcctagccccatccctccccatgaggggccaagacactgcctaaggtgtgggagggactggctgagattgcagcccatggtaggagctggaccaactgtatatagttttcaataaactttttccttttctgttcaaaaaaaaaaaaaa

SEQ ID NO: 56 - DNA, 438 bp, Homo sapiens
atggactcaggcactgtcctctttgaaatcaagaagcccccagtctcagaacggttgcccatcaaccggcgggacctggaccccaatgctgggcgctttgtccgctaccagttcacgcctgccttcctccgcctgaggcaggtgggagccacggtggagttcacagtgggagacaagcctgtcaacaacttccgcatgatcgagaggcactacttccgcaaccagctactcaaaagcttcgacttccactttggcttctgcatccccagcagcaagaacacctgcgagcacatttacgacttcccccctctctccgaggagctgatcagcgagatgatccgccacccgtatgagacccagtctgacagcttctacttcgtggatgaccggctggtgatgcacaataaagcagactattcctacagcgggacaccctga

SEQ ID NO: 57 - protein, 145 aa, Homo sapiens; identical to SEQ ID NO: 45

SEQ ID NO: 58 - DNA, 24 bp, Artificial
  Primer
aggactatcatctgatgccagagc

SEQ ID NO: 59 - DNA, 23 bp, Artificial
  Primer
tctgccacaagctgtacatctca

SEQ ID NO: 60 - DNA, 27 bp, Artificial
  Primer
agggagtttctaacaatgctgggaaca

SEQ ID NO: 61 - DNA, 27 bp, Artificial
  Primer
ctgctcctctgacttcacattcagctc

SEQ ID NO: 62 - DNA, 27 bp, Artificial
  Primer
aggctcaggagttcgaggtgacatgaa

SEQ ID NO: 63 - DNA, 27 bp, Artificial
  Primer
ggaggaccagcctcctttctacttgat

SEQ ID NO: 64 - DNA, 21 bp, Artificial
  Primer
cgtgcgtgacatcaaagagaa

SEQ ID NO: 65 - DNA, 20 bp, Artificial
  Primer
tggatgccacaggattccat

SEQ ID NO: 66 - DNA, 35 bp, Artificial
  Primer
aaaatcgatatggtggaggacggcgcggaggagct

SEQ ID NO: 67 - DNA, 35 bp, Artificial
  Primer
aaagcggccgcgaagcgcctatgcttgtaccagat

SEQ ID NO: 68 - DNA, 28 bp, Artificial
  Primer
tcccgggatgagctgaatgtgaagtcag

SEQ ID NO: 69 - DNA, 31 bp, Artificial
  Primer
tgtcgacttagatggtgagaagagggatgca

SEQ ID NO: 70 - DNA, 38 bp, Artificial
  Primer
gggctcgagatgaaggtgaagaaaggcggcggcgggac

SEQ ID NO: 71 - DNA, 38 bp, Artificial
  Primer
ggggcggccgctcagggtgtcccactgtaggaatagtc

SEQ ID NO: 72 - DNA, 36 bp, Artificial
  Primer
gggctcgagatgcagatcttcgtgaagaccctgacc

SEQ ID NO: 73 - DNA, 41 bp, Artificial
  Primer
ggggcggccgcttagccacctctcaggcgaaggaccaggtg

SEQ ID NO: 74 - DNA, 38 bp, Artificial
  Primer
gggctcgagatcccgggatgagctgaatgtgaagtcag

SEQ ID NO: 75 - DNA, 33 bp, Artificial
  Primer
tgtcgacttagatggtgagaagagggatgcagc

SEQ ID NO: 76 - DNA, 37 bp, Artificial
  Primer
gaattcgccaccatggtggaggacggcgcggaggagc

SEQ ID NO: 77 - DNA, 22 bp, Artificial
  Primer
ctttgatgctctgcagctgcag

SEQ ID NO: 78 - DNA, 35 bp, Artificial
  Primer
gggaattcatggtggaggacggcgcggaggagctg

SEQ ID NO: 79 - DNA, 34 bp, Artificial
  Primer
ggctcgaggaaagctggcaggtggggccggcgct

SEQ ID NO: 80 - DNA, 35 bp, Artificial
  Primer
tgaattcatgaaggtgaagaaaggcggcggcggga

SEQ ID NO: 81 - DNA, 34 bp, Artificial
  Primer
tgtcgactcagggtgtcccactgtaggaatagtc

SEQ ID NO: 82 - DNA, 25 bp, Artificial
  Primer
caccgagtttcttgtagccaccagc

SEQ ID NO: 83 - DNA, 25 bp, Artificial
  Primer
aaacgctggtggctacaagaaactc

SEQ ID NO: 84 - DNA, 25 bp, Artificial
  Primer
caccgactggcagtctcctccgatg

SEQ ID NO: 85 - DNA, 25 bp, Artificial
  Primer
aaaccatcggaggagactgccagtc